European Patent Application EP 4 368 638 A2, published May 15, 2024. Title: A PEPTIDE USED FOR IMMUNOTHERAPEUTICS. Applicant: (주)쓰리에이치바이오. Application US 17/823,180, filed August 30, 2022. The sequence listing filed with the application follows.

SEQUENCE LISTING (309 sequences)

SEQ ID NO: 1 - protein, 11 aa, synthetic construct
  SITE 2: note = 2nd amino acid(Xaa) is L-cyclohexylalanins.
  source 1..11: note = Th epitope
KXVAAWTLKAA

SEQ ID NO: 2 - protein, 13 aa, synthetic construct
  source 1..13: note = Th epitope
PKYVKQNTLKLAT

SEQ ID NO: 3 - protein, 15 aa, synthetic construct
  source 1..15: note = Th epitope
ILMQYIKANSKFIGI

SEQ ID NO: 4 - protein, 15 aa, synthetic construct
  source 1..15: note = Th epitope
QSIALSSLMVAQAIP

SEQ ID NO: 5 - protein, 32 aa, synthetic construct
  source 1..32: note = Th epitope
ILMQYIKANSKFIGIPMGLPQSIALSSLMVAQ

SEQ ID NO: 6 - protein, 15 aa, synthetic construct
  source 1..15: note = B cell epitope
RNVPPIFNDVYWIAF

SEQ ID NO: 7 - protein, 15 aa, synthetic construct
  source 1..15: note = B cell epitope
CRFRGLISLSQVYLS

SEQ ID NO: 8 - protein, 20 aa, synthetic construct
  source 1..20: note = B cell epitope
KTTKQSFDLSVKAQYKKNKH

SEQ ID NO: 9 - protein, 11 aa, synthetic construct
  source 1..11: note = B cell epitope
RNVPPIFNDVY

SEQ ID NO: 10 - protein, 11 aa, synthetic construct
  source 1..11: note = B cell epitope
CRFRGLISLSQ

SEQ ID NO: 11 - protein, 12 aa, synthetic construct
  source 1..12: note = B cell epitope
KTTKQSFDLSVK

SEQ ID NO: 12 - protein, 12 aa, synthetic construct
  source 1..12: note = B cell epitope
RNVPPIFNDVYW

SEQ ID NO: 13 - protein, 12 aa, synthetic construct
  source 1..12: note = B cell epitope
CRFRGLISLSQV

SEQ ID NO: 14 - protein, 17 aa, synthetic construct
  source 1..17: note = B cell epitope
KTTKQSFDLSVKAQYKK

SEQ ID NO: 15 - protein, 13 aa, synthetic construct
  source 1..13: note = B cell epitope
RNVPPIFNDVYWI

SEQ ID NO: 16 - protein, 13 aa, synthetic construct
  source 1..13: note = B cell epitope
CRFRGLISLSQVY

SEQ ID NO: 17 - protein, 18 aa, synthetic construct
  source 1..18: note = B cell epitope
KTTKQSFDLSVKAQYKKN

SEQ ID NO: 18 - protein, 11 aa, synthetic construct
  source 1..11: note = B cell epitope
PIFNDVYWIAF

SEQ ID NO: 19 - protein, 11 aa, synthetic construct
  source 1..11: note = B cell epitope
GLISLSQVYLS

SEQ ID NO: 20 - protein, 16 aa, synthetic construct
  source 1..16: note = B cell epitope
QSFDLSVKAQYKKNKH

SEQ ID NO: 21 - protein, 12 aa, synthetic construct
  source 1..12: note = B cell epitope
PPIFNDVYWIAF

SEQ ID NO: 22 - protein, 12 aa, synthetic construct
  source 1..12: note = B cell epitope
RGLISLSQVYLS

SEQ ID NO: 23 - protein, 17 aa, synthetic construct
  source 1..17: note = B cell epitope
KQSFDLSVKAQYKKNKH

SEQ ID NO: 24 - protein, 13 aa, synthetic construct
  source 1..13: note = B cell epitope
VPPIFNDVYWIAF

SEQ ID NO: 25 - protein, 13 aa, synthetic construct
  source 1..13: note = B cell epitope
FRGLISLSQVYLS

SEQ ID NO: 26 - protein, 18 aa, synthetic construct
  source 1..18: note = B cell epitope
TKQSFDLSVKAQYKKNKH

SEQ ID NO: 27 - protein, 13 aa, synthetic construct
  source 1..13: note = B cell epitope
NVPPIFNDVYWIA

SEQ ID NO: 28 - protein, 13 aa, synthetic construct
  source 1..13: note = B cell epitope
RFRGLISLSQVYL

SEQ ID NO: 29 - protein, 16 aa, synthetic construct
  source 1..16: note = B cell epitope
TKQSFDLSVKAQYKKN

SEQ ID NO: 30 - protein, 11 aa, synthetic construct
  source 1..11: note = B cell epitope
VPPIFNDVYWI

SEQ ID NO: 31 - protein, 11 aa, synthetic construct
  source 1..11: note = B cell epitope
FRGLISLSQVY

SEQ ID NO: 32 - protein, 16 aa, synthetic construct
  source 1..16: note = B cell epitope
TKQSFDLSVKAQYKKN

SEQ ID NO: 33 - protein, 9 aa, synthetic construct
  source 1..9: note = B cell epitope
PPIFNDVYW

SEQ ID NO: 34 - protein, 9 aa, synthetic construct
  source 1..9: note = B cell epitope
RGLISLSQV

SEQ ID NO: 35 - protein, 14 aa, synthetic construct
  source 1..14: note = B cell epitope
KQSFDLSVKAQYKK

SEQ ID NO: 36-39 - skipped (4 entries)

SEQ ID NO: 40 - protein, 4 aa, synthetic construct
  source 1..4: note = B cell epitope
RNVP

SEQ ID NO: 41 - protein, 4 aa, synthetic construct
  source 1..4: note = B cell epitope
WIAF

SEQ ID NO: 42-45 - skipped (4 entries)

SEQ ID NO: 46 - protein, 4 aa, synthetic construct
  source 1..4: note = B cell epitope
CRFR

SEQ ID NO: 47 - protein, 4 aa, synthetic construct
  source 1..4: note = B cell epitope
VYLS

SEQ ID NO: 48-51 - skipped (4 entries)

SEQ ID NO: 52 - protein, 15 aa, synthetic construct
  source 1..15: note = Auxiliary part
GSHHHHHHGSDDDDK

SEQ ID NO: 53 - protein, 6 aa, synthetic construct
  source 1..6: note = Auxiliary part
HHHHHH

SEQ ID NO: 54 - protein, 20 aa, synthetic construct
  source 1..20: note = His-tag sequence
MRGSHHHHHHGSDDDDKIVD

SEQ ID NO: 55 - protein, 13 aa, synthetic construct
  source 1..13: note = Linker peptide
GGGGSGGGGGGSS

SEQ ID NO: 56 - protein, 30 aa, synthetic construct
  source 1..30: note = Unit peptide
  SITE 17: note = 17th aminoacid(Xaa) is a D-form alanine.
  SITE 19: note = 19th amino acid(Xaa) is L-cyclohexylalanins.
  SITE 29: note = 29th amino acid(Xaa) is a D-form alanine.
  SITE 30: note = 30th amino acid(Xaa) is a 6-aminohexanoic acid.
  SITE 16: note = 16th amino acid(Xaa) is a 6-aminohexanoic acid.
RNVPPIFNDVYWIAFXXKXVAAWTLKAAXX

SEQ ID NO: 57 - protein, 30 aa, synthetic construct
  SITE 1: note = 1st amino acid(Xaa) is a 6-aminohexanoic acid.
  source 1..30: note = Unit peptide
  SITE 2: note = 2nd aminoacid(Xaa) is a D-form alanine.
  SITE 4: note = 4th amino acid(Xaa) isL-cyclohexylalanins.
  SITE 14: note = 14th amino acid(Xaa) is a D-form alanine.
  SITE 15: note = 15th amino acid(Xaa) is a 6-aminohexanoic acid.
XXKXVAAWTLKAAXXRNVPPIFNDVYWIAF

SEQ ID NO: 58 - protein, 30 aa, synthetic construct
  SITE 16: note = 16th amino acid(Xaa) is a 6-aminohexanoic acid.
  source 1..30: note = Unit peptide
  SITE 17: note = 17th aminoacid(Xaa) is a D-form alanine.
  SITE 19: note = 19th amino acid(Xaa) isL-cyclohexylalanins.
  SITE 29: note = 29th amino acid(Xaa) is a D-form alanine.
  SITE 30: note = 30th amino acid(Xaa) is a 6-aminohexanoic acid.
CRFRGLISLSQVYLSXXKXVAAWTLKAAXX

SEQ ID NO: 59 - protein, 30 aa, synthetic construct
  SITE 1: note = 1st amino acid(Xaa) is a 6-aminohexanoic acid.
  source 1..30: note = Unit peptide
  SITE 2: note = 2nd aminoacid(Xaa) is a D-form alanine.
  SITE 4: note = 4th amino acid(Xaa) isL-cyclohexylalanins.
  SITE 14: note = 14th amino acid(Xaa) is a D-form alanine.
  SITE 15: note = 15th amino acid(Xaa) is a 6-aminohexanoic acid.
XXKXVAAWTLKAAXXCRFRGLISLSQVYLS

SEQ ID NO: 60 - protein, 35 aa, synthetic construct
  SITE 21: note = 21st amino acid(Xaa) is a 6-aminohexanoic acid.
  source 1..35: note = Unit peptide
  SITE 22: note = 22nd aminoacid(Xaa) is a D-form alanine.
  SITE 24: note = 24th amino acid(Xaa) isL-cyclohexylalanins.
  SITE 34: note = 34th amino acid(Xaa) is a D-form alanine.
  SITE 35: note = 35th amino acid(Xaa) is a 6-aminohexanoic acid.
KTTKQSFDLSVKAQYKKNKHXXKXVAAWTLKAAXX

SEQ ID NO: 61 - protein, 35 aa, synthetic construct
  SITE 1: note = 1st amino acid(Xaa) is a 6-aminohexanoic acid.
  source 1..35: note = Unit peptide
  SITE 2: note = 2nd aminoacid(Xaa) is a D-form alanine.
  SITE 4: note = 4th amino acid(Xaa) is L-cyclohexylalanins.
  SITE 14: note = 14th amino acid(Xaa) is a D-form alanine.
  SITE 15: note = 15th amino acid(Xaa) is a 6-aminohexanoic acid.
XXKXVAAWTLKAAXXKTTKQSFDLSVKAQYKKNKH

SEQ ID NO: 62 - protein, 26 aa, synthetic construct
  SITE 17: note = 17th amino acid(Xaa) is L-cyclohexylalanins.
  source 1..26: note = Unit peptide
RNVPPIFNDVYWIAFKXVAAWTLKAA

SEQ ID NO: 63 - protein, 26 aa, synthetic construct
  SITE 2: note = 2nd amino acid(Xaa) is L-cyclohexylalanins.
  source 1..26: note = Unit peptide
KXVAAWTLKAARNVPPIFNDVYWIAF

SEQ ID NO: 64 - protein, 22 aa, synthetic construct
  SITE 13: note = 13rd amino acid(Xaa) is L-cyclohexylalanins.
  source 1..22: note = Unit peptide
RNVPPIFNDVYKXVAAWTLKAA

SEQ ID NO: 65 - protein, 22 aa, synthetic construct
  SITE 13: note = 13rd amino acid(Xaa) is L-cyclohexylalanins.
  source 1..22: note = Unit peptide
PIFNDVYWIAFKXVAAWTLKAA

SEQ ID NO: 66 - protein, 20 aa, synthetic construct
  SITE 11: note = 11st amino acid(Xaa) is L-cyclohexylalanins.
  source 1..20: note = Unit peptide
PPIFNDVYWKXVAAWTLKAA

SEQ ID NO: 67 - protein, 32 aa, synthetic construct
  SITE 17: note = 17th amino acid(Xaa) is L-cyclohexylalanins.
  source 1..32: note = Unit peptide
RNVPPIFNDVYWIAFKXVAAWTLKAAHHHHHH

SEQ ID NO: 68 - protein, 45 aa, synthetic construct
  SITE 16: note = 16th amino acid(Xaa) is a 6-aminohexanoic acid.
  source 1..45: note = Unit peptide
  SITE 17: note = 17th aminoacid(Xaa) is a D-form alanine.
  SITE 19: note = 19th amino acid(Xaa) is L-cyclohexylalanins.
  SITE 29: note = 29th amino acid(Xaa) is a D-form alanine.
  SITE 30: note = 30th amino acid(Xaa) is a 6-aminohexanoic acid.
RNVPPIFNDVYWIAFXXKXVAAWTLKAAXXGSHHHHHHGSDDDDK

SEQ ID NO: 69 - protein, 45 aa, synthetic construct
  SITE 16: note = 16th amino acid(Xaa) is a 6-aminohexanoic acid.
  source 1..45: note = Unit peptide
  SITE 17: note = 17th aminoacid(Xaa) is a D-form alanine.
  SITE 19: note = 19th amino acid(Xaa) isL-cyclohexylalanins.
  SITE 29: note = 29th amino acid(Xaa) is a D-form alanine.
  SITE 30: note = 30th amino acid(Xaa) is a 6-aminohexanoic acid.
GSHHHHHHGSDDDDKXXKXVAAWTLKAAXXRNVPPIFNDVYWIAF

SEQ ID NO: 70 - protein, 45 aa, synthetic construct
  SITE 31: note = 31st amino acid(Xaa) is a 6-aminohexanoic acid.
  source 1..45: note = Unit peptide
  SITE 32: note = 32nd aminoacid(Xaa) is a D-form alanine.
  SITE 34: note = 34th amino acid(Xaa) isL-cyclohexylalanins.
  SITE 44: note = 44th amino acid(Xaa) is a D-form alanine.
  SITE 45: note = 45th amino acid(Xaa) is a 6-aminohexanoic acid.
RNVPPIFNDVYWIAFGSHHHHHHGSDDDDKXXKXVAAWTLKAAXX

SEQ ID NO: 71 - protein, 45 aa, synthetic construct
  SITE 16: note = 16th amino acid(Xaa) is a 6-aminohexanoic acid.
  source 1..45: note = Unit peptide
  SITE 19: note = 19th amino acid(Xaa) isL-cyclohexylalanins.
  SITE 29: note = 29th amino acid(Xaa) is a D-form alanine.
  SITE 30: note = 30th amino acid(Xaa) is a 6-aminohexanoic acid.
  SITE 17: note = 17th aminoacid(Xaa) is a D-form alanine.
GSHHHHHHGSDDDDKXXKXVAAWTLKAAXXCRFRGLISLSQVYLS

SEQ ID NO: 72 - protein, 45 aa, synthetic construct
  source 1..45: note = Unit peptide
  SITE 31: note = 31st amino acid(Xaa) is a 6-aminohexanoic acid.
  SITE 32: note = 32nd aminoacid(Xaa) is a D-form alanine.
  SITE 34: note = 34th amino acid(Xaa) isL-cyclohexylalanins.
  SITE 44: note = 44th amino acid(Xaa) is a D-form alanine.
  SITE 45: note = 45th amino acid(Xaa) is a 6-aminohexanoic acid.
GSHHHHHHGSDDDDKCRFRGLISLSQVYLSXXKXVAAWTLKAAXX

SEQ ID NO: 73 - protein, 45 aa, synthetic construct
  source 1..45: note = Unit peptide
  SITE 16: note = 16th amino acid(Xaa) is a 6-aminohexanoic acid.
  SITE 17: note = 17th aminoacid(Xaa) is a D-form alanine.
  SITE 19: note = 19th amino acid(Xaa) isL-cyclohexylalanins.
  SITE 29: note = 29th amino acid(Xaa) is a D-form alanine.
  SITE 30: note = 30th amino acid(Xaa) is a 6-aminohexanoic acid.
CRFRGLISLSQVYLSXXKXVAAWTLKAAXXGSHHHHHHGSDDDDK

SEQ ID NO: 74 - protein, 50 aa, synthetic construct
  source 1..50: note = Unit peptide
  SITE 16: note = 16th amino acid(Xaa) is a 6-aminohexanoic acid.
  SITE 17: note = 17th aminoacid(Xaa) is a D-form alanine.
  SITE 19: note = 19th amino acid(Xaa) isL-cyclohexylalanins.
  SITE 29: note = 29th amino acid(Xaa) is a D-form alanine.
  SITE 30: note = 30th amino acid(Xaa) is a 6-aminohexanoic acid.
GSHHHHHHGSDDDDKXXKXVAAWTLKAAXXKTTKQSFDLSVKAQYKKNKH

SEQ ID NO: 75 - protein, 50 aa, synthetic construct
  source 1..50: note = Unit peptide
  SITE 36: note = 36th amino acid(Xaa) is a 6-aminohexanoic acid.
  SITE 37: note = 37th aminoacid(Xaa) is a D-form alanine.
  SITE 39: note = 39th amino acid(Xaa) isL-cyclohexylalanins.
  SITE 49: note = 49th amino acid(Xaa) is a D-form alanine.
  SITE 50: note = 50th amino acid(Xaa) is a 6-aminohexanoic acid.
GSHHHHHHGSDDDDKKTTKQSFDLSVKAQYKKNKHXXKXVAAWTLKAAXX

SEQ ID NO: 76 - protein, 50 aa, synthetic construct
  source 1..50: note = Unit peptide
  SITE 21: note = 21st amino acid(Xaa) is a 6-aminohexanoic acid.
  SITE 22: note = 22nd aminoacid(Xaa) is a D-form alanine.
  SITE 24: note = 24th amino acid(Xaa) is L-cyclohexylalanins.
  SITE 34: note = 34th amino acid(Xaa) is a D-form alanine.
  SITE 35: note = 35th amino acid(Xaa) is a 6-aminohexanoic acid.
KTTKQSFDLSVKAQYKKNKHXXKXVAAWTLKAAXXGSHHHHHHGSDDDDK

SEQ ID NO: 77 - protein, 50 aa, synthetic construct
  source 1..50: note = Unit peptide
  SITE 36: note = 36th amino acid(Xaa) is a 6-aminohexanoic acid.
  SITE 37: note = 37th aminoacid(Xaa) is a D-form alanine.
  SITE 39: note = 39th amino acid(Xaa) isL-cyclohexylalanins.
  SITE 49: note = 49th amino acid(Xaa) is a D-form alanine.
  SITE 50: note = 50th amino acid(Xaa) is a 6-aminohexanoic acid.
MRGSHHHHHHGSDDDDKIVDRNVPPIFNDVYWIAFXXKXVAAWTLKAAXX

SEQ ID NO: 78 - protein, 65 aa, synthetic construct
  source 1..65: note = Unit peptide
  SITE 51: note = 51st amino acid(Xaa) is a 6-aminohexanoic acid.
  SITE 52: note = 52nd aminoacid(Xaa) is a D-form alanine.
  SITE 54: note = 54th amino acid(Xaa) is L-cyclohexylalanins.
  SITE 64: note = 64th amino acid(Xaa) is a D-form alanine.
  SITE 65: note = 65th amino acid(Xaa) is a 6-aminohexanoic acid.
MRGSHHHHHHGSDDDDKIVDGSHHHHHHGSDDDDKRNVPPIFNDVYWIAFXXKXVAAWTLKAAXX

SEQ ID NO: 79 - protein, 65 aa, synthetic construct
  source 1..65: note = Unit peptide
  SITE 36: note = 36th amino acid(Xaa) is a 6-aminohexanoic acid.
  SITE 37: note = 37th aminoacid(Xaa) is a D-form alanine.
  SITE 39: note = 39th amino acid(Xaa) is L-cyclohexylalanins.
  SITE 49: note = 49th amino acid(Xaa) is a D-form alanine.
  SITE 50: note = 50th amino acid(Xaa) is a 6-aminohexanoic acid.
MRGSHHHHHHGSDDDDKIVDRNVPPIFNDVYWIAFXXKXVAAWTLKAAXXGSHHHHHHGSDDDDK

SEQ ID NO: 80 - protein, 30 aa, synthetic construct
  source 1..30: note = Unit peptide
RNVPPIFNDVYWIAFILMQYIKANSKFIGI

SEQ ID NO: 81 - protein, 47 aa, synthetic construct
  source 1..47: note = Unit peptide
RNVPPIFNDVYWIAFILMQYIKANSKFIGIPMGLPQSIALSSLMVAQ

SEQ ID NO: 82 - protein, 32 aa, synthetic construct
  source 1..32: note = Unit peptide
  SITE 17: note = 17th amino acid(Xaa) is a 6-aminohexanoic acid.
  SITE 18: note = 18th amino acid(Xaa) is a D-form alanine.
  SITE 20: note = 20th amino acid(Xaa) is L-cyclohexylalanins.
  SITE 30: note = 30th amino acid(Xaa) is a D-form alanine.
  SITE 31: note = 31st amino acid(Xaa) is a 6-aminohexanoic acid.
CRNVPPIFNDVYWIAFXXKXVAAWTLKAAXXC

SEQ ID NO: 83 - protein, 45 aa, synthetic construct
  source 1..45: note = Unit peptide
  SITE 31: note = 31st amino acid(Xaa) is a 6-aminohexanoic acid.
  SITE 32: note = 32nd amino acid(Xaa) is a D-form alanine.
  SITE 34: note = 34th amino acid(Xaa) is L-cyclohexylalanins.
  SITE 44: note = 44th amino acid(Xaa) is a D-form alanine.
  SITE 45: note = 45th amino acid(Xaa) is a 6-aminohexanoic acid.
RNVPPIFNDVYWIAFRNVPPIFNDVYWIAFXXKXVAAWTLKAAXX

SEQ ID NO: 84 - protein, 45 aa, synthetic construct
  source 1..45: note = Unit peptide
  SITE 31: note = 31st amino acid(Xaa) is a 6-aminohexanoic acid.
  SITE 32: note = 32nd amino acid(Xaa) is a D-form alanine.
  SITE 34: note = 34th amino acid(Xaa) is L-cyclohexylalanins.
  SITE 44: note = 44th amino acid(Xaa) is a D-form alanine.
  SITE 45: note = 45th amino acid(Xaa) is a 6-aminohexanoic acid.
RNVPPIFNDVYWIAFCRFRGLISLSQVYLSXXKXVAAWTLKAAXX

SEQ ID NO: 85 - protein, 50 aa, synthetic construct
  source 1..50: note = Unit peptide
  SITE 36: note = 36th amino acid(Xaa) is a 6-aminohexanoic acid.
  SITE 37: note = 37th amino acid(Xaa) is a D-form alanine.
  SITE 39: note = 39th amino acid(Xaa) is L-cyclohexylalanins.
  SITE 49: note = 49th amino acid(Xaa) is a D-form alanine.
  SITE 50: note = 50th amino acid(Xaa) is a 6-aminohexanoic acid.
RNVPPIFNDVYWIAFKTTKQSFDLSVKAQYKKNKHXXKXVAAWTLKAAXX

SEQ ID NO: 86 - protein, 45 aa, synthetic construct
  source 1..45: note = Unit peptide
  SITE 31: note = 31st amino acid(Xaa) is a 6-aminohexanoic acid.
  SITE 32: note = 32nd amino acid(Xaa) is a D-form alanine.
  SITE 34: note = 34th amino acid(Xaa) is L-cyclohexylalanins.
  SITE 44: note = 44th amino acid(Xaa) is a D-form alanine.
  SITE 45: note = 45th amino acid(Xaa) is a 6-aminohexanoic acid.
CRFRGLISLSQVYLSRNVPPIFNDVYWIAFXXKXVAAWTLKAAXX

SEQ ID NO: 87 - protein, 45 aa, synthetic construct
  source 1..45: note = Unit peptide
  SITE 31: note = 31st amino acid(Xaa) is a 6-aminohexanoic acid.
  SITE 32: note = 32nd amino acid(Xaa) is a D-form alanine.
  SITE 34: note = 34th amino acid(Xaa) is L-cyclohexylalanins.
  SITE 44: note = 44th amino acid(Xaa) is a D-form alanine.
  SITE 45: note = 45th amino acid(Xaa) is a 6-aminohexanoic acid.
CRFRGLISLSQVYLSCRFRGLISLSQVYLSXXKXVAAWTLKAAXX

SEQ ID NO: 88 - protein, 50 aa, synthetic construct
  source 1..50: note = Unit peptide
  SITE 36: note = 36th amino acid(Xaa) is a 6-aminohexanoic acid.
  SITE 37: note = 37th amino acid(Xaa) is a D-form alanine.
  SITE 39: note = 39th amino acid(Xaa) is L-cyclohexylalanins.
  SITE 49: note = 49th amino acid(Xaa) is a D-form alanine.
  SITE 50: note = 50th amino acid(Xaa) is a 6-aminohexanoic acid.
CRFRGLISLSQVYLSKTTKQSFDLSVKAQYKKNKHXXKXVAAWTLKAAXX

SEQ ID NO: 89 - protein, 50 aa, synthetic construct
  source 1..50: note = Unit peptide
  SITE 36: note = 36th amino acid(Xaa) is a 6-aminohexanoic acid.
  SITE 37: note = 37th amino acid(Xaa) is a D-form alanine.
  SITE 39: note = 39th amino acid(Xaa) is L-cyclohexylalanins.
  SITE 49: note = 49th amino acid(Xaa) is a D-form alanine.
  SITE 50: note = 50th amino acid(Xaa) is a 6-aminohexanoic acid.
KTTKQSFDLSVKAQYKKNKHRNVPPIFNDVYWIAFXXKXVAAWTLKAAXX

SEQ ID NO: 90 - protein, 50 aa, synthetic construct
  source 1..50: note = Unit peptide
  SITE 36: note = 36th amino acid(Xaa) is a 6-aminohexanoic acid.
  SITE 37: note = 37th amino acid(Xaa) is a D-form alanine.
  SITE 39: note = 39th amino acid(Xaa) is L-cyclohexylalanins.
  SITE 49: note = 49th amino acid(Xaa) is a D-form alanine.
  SITE 50: note = 50th amino acid(Xaa) is a 6-aminohexanoic acid.
KTTKQSFDLSVKAQYKKNKHCRFRGLISLSQVYLSXXKXVAAWTLKAAXX

SEQ ID NO: 91 - protein, 55 aa, synthetic construct
  source 1..55: note = Unit peptide
  SITE 41: note = 41st amino acid(Xaa) is a 6-aminohexanoic acid.
  SITE 42: note = 42nd amino acid(Xaa) is a D-form alanine.
  SITE 44: note = 44th amino acid(Xaa) is L-cyclohexylalanins.
  SITE 54: note = 54th amino acid(Xaa) is a D-form alanine.
  SITE 55: note = 55th amino acid(Xaa) is a 6-aminohexanoic acid.
KTTKQSFDLSVKAQYKKNKHKTTKQSFDLSVKAQYKKNKHXXKXVAAWTLKAAXX

SEQ ID NO: 92 - protein, 41 aa, synthetic construct
  source 1..41: note = Unit peptide
  SITE 32: note = 32nd amino acid(Xaa) is L-cyclohexylalanins.
RNVPPIFNDVYWIAFCRFRGLISLSQVYLSKXVAAWTLKAA

SEQ ID NO: 93 - protein, 33 aa, synthetic construct
  source 1..33: note = Unit peptide
  SITE 24: note = 24th amino acid(Xaa) is L-cyclohexylalanins.
PIFNDVYWIAFGLISLSQVYLSKXVAAWTLKAA

SEQ ID NO: 94 - protein, 33 aa, synthetic construct
  source 1..33: note = Unit peptide
  SITE 24: note = 24th amino acid(Xaa) is L-cyclohexylalanins.
RNVPPIFNDVYCRFRGLISLSQKXVAAWTLKAA

SEQ ID NO: 95 - protein, 33 aa, synthetic construct
  source 1..33: note = Unit peptide
  SITE 24: note = 24th amino acid(Xaa) is L-cyclohexylalanins.
PIFNDVYWIAFCRFRGLISLSQKXVAAWTLKAA

SEQ ID NO: 96 - protein, 29 aa, synthetic construct
  source 1..29: note = Unit peptide
  SITE 20: note = 20th amino acid(Xaa) is L-cyclohexylalanins.
PPIFNDVYWRGLISLSQVKXVAAWTLKAA

SEQ ID NO: 97 - protein, 47 aa, synthetic construct
  source 1..47: note = Unit peptide
  SITE 32: note = 32nd amino acid(Xaa) is L-cyclohexylalanins.
RNVPPIFNDVYWIAFCRFRGLISLSQVYLSKXVAAWTLKAAHHHHHH

SEQ ID NO: 98 - protein, 65 aa, synthetic construct
  source 1..65: note = Unit peptide
  SITE 51: note = 51st amino acid(Xaa) is a 6-aminohexanoic acid.
  SITE 52: note = 52nd amino acid(Xaa) is a D-form alanine.
  SITE 54: note = 54th amino acid(Xaa) is L-cyclohexylalanins.
  SITE 64: note = 64th amino acid(Xaa) is a D-form alanine.
  SITE 65: note = 65th amino acid(Xaa) is a 6-aminohexanoic acid.
MRGSHHHHHHGSDDDDKIVDRNVPPIFNDVYWIAFCRFRGLISLSQVYLSXXKXVAAWTLKAAXX

SEQ ID NO: 99 - protein, 63 aa, synthetic construct
  source 1..63: note = Unit peptide
  SITE 51: note = 51st amino acid(Xaa) is a 6-aminohexanoic acid.
  SITE 52: note = 52nd amino acid(Xaa) is a D-form alanine.
  SITE 54: note = 54th amino acid(Xaa) is L-cyclohexylalanins.
MRGSHHHHHHGSDDDDKIVDRNVPPIFNDVYWIAFCRFRGLISLSQVYLSXXKXVAAWTLKAA

SEQ ID NO: 100 - protein, 43 aa, synthetic construct
  source 1..43: note = Unit peptide
  SITE 31: note = 31st amino acid(Xaa) is a 6-aminohexanoic acid.
  SITE 32: note = 32nd amino acid(Xaa) is a D-form alanine.
  SITE 34: note = 34th amino acid(Xaa) is L-cyclohexylalanins.
RNVPPIFNDVYWIAFCRFRGLISLSQVYLSXXKXVAAWTLKAA

SEQ ID NO: 101 - protein, 76 aa, synthetic construct
  source 1..76: note = Unit peptide
  SITE 64: note = 64th amino acid(Xaa) is a 6-aminohexanoic acid.
  SITE 65: note = 65th amino acid(Xaa) is a D-form alanine.
  SITE 67: note = 67th amino acid(Xaa) is L-cyclohexylalanins.
MRGSHHHHHHGSDDDDKIVDRNVPPIFNDVYWIAFGGGGSGGGGGGSSRNVPPIFNDVYWIAFXXKXVAAWTLKAA

SEQ ID NO: 102 - protein, 56 aa, synthetic construct
  source 1..56: note = Unit peptide
  SITE 44: note = 44th amino acid(Xaa) is a 6-aminohexanoic acid.
  SITE 45: note = 45th amino acid(Xaa) is a D-form alanine.
  SITE 47: note = 47th amino acid(Xaa) is L-cyclohexylalanins.
RNVPPIFNDVYWIAFGGGGSGGGGGGSSRNVPPIFNDVYWIAFXXKXVAAWTLKAA

SEQ ID NO: 103 - protein, 58 aa, synthetic construct
  source 1..58: note = Unit peptide
  SITE 44: note = 44th amino acid(Xaa) is a 6-aminohexanoic acid.
  SITE 45: note = 45th amino acid(Xaa) is a D-form alanine.
  SITE 47: note = 47th amino acid(Xaa) is L-cyclohexylalanins.
  SITE 57: note = 57th amino acid(Xaa) is a D-form alanine.
  SITE 58: note = 58th amino acid(Xaa) is a 6-aminohexanoic acid.
RNVPPIFNDVYWIAFGGGGSGGGGGGSSRNVPPIFNDVYWIAFXXKXVAAWTLKAAXX

SEQ ID NO: 104 - protein, 45 aa, synthetic construct
  source 1..45: note = Unit peptide
RNVPPIFNDVYWIAFRNVPPIFNDVYWIAFILMQYIKANSKFIGI

SEQ ID NO: 105 - protein, 62 aa, synthetic construct
  source 1..62: note = Unit peptide
RNVPPIFNDVYWIAFRNVPPIFNDVYWIAFILMQYIKANSKFIGIPMGLPQSIALSSLMVAQ

SEQ ID NO: 106 - protein, 47 aa, synthetic construct
  source 1..47: note = Unit peptide
  SITE 32: note = 32nd amino acid(Xaa) is a 6-aminohexanoic acid.
  SITE 33: note = 33rd amino acid(Xaa) is a D-form alanine.
  SITE 35: note = 35th amino acid(Xaa) is L-cyclohexylalanins.
  SITE 45: note = 45th amino acid(Xaa) is a D-form alanine.
  SITE 46: note = 46th amino acid(Xaa) is a 6-aminohexanoic acid.
CRNVPPIFNDVYWIAFCRFRGLISLSQVYLSXXKXVAAWTLKAAXXC

SEQ ID NO: 107 - protein, 45 aa, synthetic construct
  source 1..45: note = Unit peptide
  SITE 16: note = 16th amino acid(Xaa) is a 6-aminohexanoic acid.
  SITE 17: note = 17th amino acid(Xaa) is a D-form alanine.
  SITE 19: note = 19th amino acid(Xaa) is L-cyclohexylalanins.
  SITE 29: note = 29th amino acid(Xaa) is a D-form alanine.
  SITE 30: note = 30th amino acid(Xaa) is a 6-aminohexanoic acid.
RNVPPIFNDVYWIAFXXKXVAAWTLKAAXXRNVPPIFNDVYWIAF

SEQ ID NO: 108 - protein, 45 aa, synthetic construct
  source 1..45: note = Unit peptide
  SITE 16: note = 16th amino acid(Xaa) is a 6-aminohexanoic acid.
  SITE 17: note = 17th amino acid(Xaa) is a D-form alanine.
  SITE 19: note = 19th amino acid(Xaa) is L-cyclohexylalanins.
  SITE 29: note = 29th amino acid(Xaa) is a D-form alanine.
  SITE 30: note = 30th amino acid(Xaa) is a 6-aminohexanoic acid.
RNVPPIFNDVYWIAFXXKXVAAWTLKAAXXCRFRGLISLSQVYLS

SEQ ID NO: 109 - protein, 50 aa, synthetic construct
  source 1..50: note = Unit peptide
  SITE 16: note = 16th amino acid(Xaa) is a 6-aminohexanoic acid.
  SITE 17: note = 17th amino acid(Xaa) is a D-form alanine.
  SITE 19: note = 19th amino acid(Xaa) is L-cyclohexylalanins.
  SITE 29: note = 29th amino acid(Xaa) is a D-form alanine.
  SITE 30: note = 30th amino acid(Xaa) is a 6-aminohexanoic acid.
RNVPPIFNDVYWIAFXXKXVAAWTLKAAXXKTTKQSFDLSVKAQYKKNKH

SEQ ID NO: 110 - protein, 45 aa, synthetic construct
  source 1..45: note = Unit peptide
  SITE 16: note = 16th amino acid(Xaa) is a 6-aminohexanoic acid.
  SITE 17: note = 17th amino acid(Xaa) is a D-form alanine.
  SITE 19: note = 19th amino acid(Xaa) is L-cyclohexylalanins.
  SITE 29: note = 29th amino acid(Xaa) is a D-form alanine.
  SITE 30: note = 30th amino acid(Xaa) is a 6-aminohexanoic acid.
CRFRGLISLSQVYLSXXKXVAAWTLKAAXXRNVPPIFNDVYWIAF

SEQ ID NO: 111 - protein, 45 aa, synthetic construct
  source 1..45: note = Unit peptide
  SITE 16: note = 16th amino acid(Xaa) is a 6-aminohexanoic acid.
  SITE 17: note = 17th amino acid(Xaa) is a D-form alanine.
  SITE 19: note = 19th amino acid(Xaa) is L-cyclohexylalanins.
  SITE 29: note = 29th amino acid(Xaa) is a D-form alanine.
  SITE 30: note = 30th amino acid(Xaa) is a 6-aminohexanoic acid.
CRFRGLISLSQVYLSXXKXVAAWTLKAAXXCRFRGLISLSQVYLS

SEQ ID NO: 112 - protein, 50 aa, synthetic construct; identical to SEQ ID NO: 109
  source 1..50: note = Unit peptide
  SITE 16: note = 16th amino acid(Xaa) is a 6-aminohexanoic acid.
  SITE 17: note = 17th amino acid(Xaa) is a D-form alanine.
  SITE 19: note = 19th amino acid(Xaa) is L-cyclohexylalanins.
  SITE 29: note = 29th amino acid(Xaa) is a D-form alanine.
  SITE 30: note = 30th amino acid(Xaa) is a 6-aminohexanoic acid.

SEQ ID NO: 113 - protein, 50 aa, synthetic construct
  source 1..50: note = Unit peptide
  SITE 21: note = 21st amino acid(Xaa) is a 6-aminohexanoic acid.
  SITE 22: note = 22nd amino acid(Xaa) is a D-form alanine.
  SITE 24: note = 24th amino acid(Xaa) is L-cyclohexylalanins.
  SITE 34: note = 34th amino acid(Xaa) is a D-form alanine.
  SITE 35: note = 35th amino acid(Xaa) is a 6-aminohexanoic acid.
KTTKQSFDLSVKAQYKKNKHXXKXVAAWTLKAAXXRNVPPIFNDVYWIAF

SEQ ID NO: 114 - protein, 50 aa, synthetic construct
  source 1..50: note = Unit peptide
  SITE 21: note = 21st amino acid(Xaa) is a 6-aminohexanoic acid.
  SITE 22: note = 22nd amino acid(Xaa) is a D-form alanine.
  SITE 24: note = 24th amino acid(Xaa) is L-cyclohexylalanins.
  SITE 34: note = 34th amino acid(Xaa) is a D-form alanine.
  SITE 35: note = 35th amino acid(Xaa) is a 6-aminohexanoic acid.
KTTKQSFDLSVKAQYKKNKHXXKXVAAWTLKAAXXCRFRGLISLSQVYLS

SEQ ID NO: 115 - protein, 55 aa, synthetic construct
  source 1..55: note = Unit peptide
  SITE 21: note = 21st amino acid(Xaa) is a 6-aminohexanoic acid.
  SITE 22: note = 22nd amino acid(Xaa) is a D-form alanine.
  SITE 24: note = 24th amino acid(Xaa) is L-cyclohexylalanins.
  SITE 34: note = 34th amino acid(Xaa) is a D-form alanine.
  SITE 35: note = 35th amino acid(Xaa) is a 6-aminohexanoic acid.
KTTKQSFDLSVKAQYKKNKHXXKXVAAWTLKAAXXKTTKQSFDLSVKAQYKKNKH

SEQ ID NO: 116 - protein, 33 aa, synthetic construct
  source 1..33: note = Unit peptide
  SITE 13: note = 13rd amino acid(Xaa) is L-cyclohexylalanins.
PIFNDVYWIAFKXVAAWTLKAACRFRGLISLSQ

SEQ ID NO: 117 - protein, 29 aa, synthetic construct
  source 1..29: note = Unit peptide
  VARIANT 11: note = Xaa can be any naturally occurring amino acid.
PPIFNDVYWKXVAAWTLKAARGLISLSQV

SEQ ID NO: 118 - protein, 65 aa, synthetic construct
  source 1..65: note = Unit peptide
  SITE 36: note = 36th amino acid(Xaa) is a 6-aminohexanoic acid.
  SITE 37: note = 37th amino acid(Xaa) is a D-form alanine.
  SITE 39: note = 39th amino acid(Xaa) is L-cyclohexylalanins.
  SITE 49: note = 49th amino acid(Xaa) is a D-form alanine.
  SITE 50: note = 50th amino acid(Xaa) is a 6-aminohexanoic acid.
MRGSHHHHHHGSDDDDKIVDRNVPPIFNDVYWIAFXXKXVAAWTLKAAXXRNVPPIFNDVYWIAF

SEQ ID NO: 119 - protein, 108 aa, synthetic construct
  source 1..108: note = Unit peptide
MRGSHHHHHHGSDDDDKIVDRNVPPIFNDVYWIAFGGGGSGGGGGGSSILMQYIKANSKFIGIPMGLPQSIALSSLMVAQGGGGSGGGGGGSSCRFRGLISLSQVYLS

SEQ ID NO: 120 - protein, 45 aa, synthetic construct
  source 1..45: note = Unit peptide
RNVPPIFNDVYWIAFILMQYIKANSKFIGICRFRGLISLSQVYLS

SEQ ID NO: 121 - protein, 45 aa, synthetic construct
  source 1..45: note = Unit peptide
  SITE 16: note = 16th amino acid(Xaa) is a 6-aminohexanoic acid.
  SITE 17: note = 17th amino acid(Xaa) is a D-form alanine.
  SITE 19: note = 19th amino acid(Xaa) is L-cyclohexylalanins.
  SITE 29: note = 29th amino acid(Xaa) is a D-form alanine.
  SITE 30: note = 30th amino acid(Xaa) is a 6-aminohexanoic acid.
RNVPPIFNDVYWIAFXPKYVKQNTLKLATXCRFRGLISLSQVYLS

SEQ ID NO: 122 - protein, 47 aa, synthetic construct
  source 1..47: note = Unit peptide
  SITE 17: note = 17th amino acid(Xaa) is a 6-aminohexanoic acid.
  SITE 18: note = 18th amino acid(Xaa) is a D-form alanine.
  SITE 20: note = 20th amino acid(Xaa) is L-cyclohexylalanins.
  SITE 30: note = 30th amino acid(Xaa) is a D-form alanine.
  SITE 31: note = 31st amino acid(Xaa) is a 6-aminohexanoic acid.
CRNVPPIFNDVYWIAFXXKXVAAWTLKAAXXRNVPPIFNDVYWIAFC

SEQ ID NO: 123 - protein, 45 aa, synthetic construct
  source 1..45: note = Unit peptide
  SITE 16: note = 16th amino acid(Xaa) is a 6-aminohexanoic acid.
  SITE 17: note = 17th amino acid(Xaa) is a D-form alanine.
  SITE 19: note = 19th amino acid(Xaa) is L-cyclohexylalanins.
  SITE 29: note = 29th amino acid(Xaa) is a D-form alanine.
  SITE 30: note = 30th amino acid(Xaa) is a 6-aminohexanoic acid.
RNVPPIFNDVYWIAFXXKXVAAWTLKAAXXILMQYIKANSKFIGI

SEQ ID NO: 124 - protein, 45 aa, synthetic construct
  source 1..45: note = Unit peptide
  SITE 16: note = 16th amino acid(Xaa) is a 6-aminohexanoic acid.
  SITE 17: note = 17th amino acid(Xaa) is a D-form alanine.
  SITE 19: note = 19th amino acid(Xaa) is L-cyclohexylalanins.
  SITE 29: note = 29th amino acid(Xaa) is a D-form alanine.
  SITE 30: note = 30th amino acid(Xaa) is a 6-aminohexanoic acid.
CRFRGLISLSQVYLSXXKXVAAWTLKAAXXILMQYIKANSKFIGI

SEQ ID NO: 125 - protein, 50 aa, synthetic construct
  source 1..50: note = Unit peptide
  SITE 21: note = 21st amino acid(Xaa) is a 6-aminohexanoic acid.
  SITE 22: note = 22nd amino acid(Xaa) is a D-form alanine.
  SITE 24: note = 24th amino acid(Xaa) is L-cyclohexylalanins.
  SITE 34: note = 34th amino acid(Xaa) is a D-form alanine.
  SITE 35: note = 35th amino acid(Xaa) is a 6-aminohexanoic acid.
KTTKQSFDLSVKAQYKKNKHXXKXVAAWTLKAAXXILMQYIKANSKFIGI

SEQ ID NO: 126 - protein, 45 aa, synthetic construct
  source 1..45: note = Unit peptide
  SITE 16: note = 16th amino acid(Xaa) is a 6-aminohexanoic acid.
  SITE 17: note = 17th amino acid(Xaa) is a D-form alanine.
  SITE 19: note = 19th amino acid(Xaa) is L-cyclohexylalanins.
  SITE 29: note = 29th amino acid(Xaa) is a D-form alanine.
  SITE 30: note = 30th amino acid(Xaa) is a 6-aminohexanoic acid.
ILMQYIKANSKFIGIXXKXVAAWTLKAAXXRNVPPIFNDVYWIAF

SEQ ID NO: 127 - protein, 45 aa, synthetic construct
  source 1..45: note = Unit peptide
  SITE 16: note = 16th amino acid(Xaa) is a 6-aminohexanoic acid.
  SITE 17: note = 17th amino acid(Xaa) is a D-form alanine.
  SITE 19: note = 19th amino acid(Xaa) is L-cyclohexylalanins.
  SITE 29: note = 29th amino acid(Xaa) is a D-form alanine.
  SITE 30: note = 30th amino acid(Xaa) is a 6-aminohexanoic acid.
ILMQYIKANSKFIGIXXKXVAAWTLKAAXXCRFRGLISLSQVYLS

SEQ ID NO: 128 - protein, 50 aa, synthetic construct
  source 1..50: note = Unit peptide
  SITE 16: note = 16th amino acid(Xaa) is a 6-aminohexanoic acid.
  SITE 17: note = 17th amino acid(Xaa) is a D-form alanine.
  SITE 19: note = 19th amino acid(Xaa) is L-cyclohexylalanins.
  SITE 29: note = 29th amino acid(Xaa) is a D-form alanine.
  SITE 30: note = 30th amino acid(Xaa) is a 6-aminohexanoic acid.
ILMQYIKANSKFIGIXXKXVAAWTLKAAXXKTTKQSFDLSVKAQYKKNKH

SEQ ID NO: 129 - protein, 33 aa, synthetic construct
  source 1..33: note = Unit peptide
  SITE 13: note = 13rd amino acid(Xaa) is L-cyclohexylalanins.
  SITE 24: note = 24th amino acid(Xaa)is L-cyclohexylalanins.
PIFNDVYWIAFKXVAAWTLKAAKXVAAWTLKAA

SEQ ID NO: 130 - protein, 31 aa, synthetic construct
  source 1..31: note = Unit peptide
  SITE 11: note = 11st amino acid(Xaa) is L-cyclohexylalanins.
  SITE 21: note = 21st amino acid(Xaa)is L-cyclohexylalanins.
PPIFNDVYWKXVAAWTLKAAKXVAAWTLKAA

SEQ ID NO: 131 - protein, 65 aa, synthetic construct
  source 1..65: note = Unit peptide
  SITE 36: note = 36th amino acid(Xaa) is a 6-aminohexanoic acid.
  SITE 37: note = 37th amino acid(Xaa) is a D-form alanine.
  SITE 39: note = 39th amino acid(Xaa) is L-cyclohexylalanins.
  SITE 49: note = 49th amino acid(Xaa) is a D-form alanine.
  SITE 50: note = 50th amino acid(Xaa) is a 6-aminohexanoic acid.
MRGSHHHHHHGSDDDDKIVDRNVPPIFNDVYWIAFXXKXVAAWTLKAAXXILMQYIKANSKFIGI

SEQ ID NO: 132 - protein, 50 aa, synthetic construct
  source 1..50: note = Unit peptide
  SITE 36: note = 36th amino acid(Xaa) is a 6-aminohexanoic acid.
  SITE 37: note = 37th amino acid(Xaa) is a D-form alanine.
  SITE 39: note = 39th amino acid(Xaa) is L-cyclohexylalanins.
  SITE 49: note = 49th amino acid(Xaa) is a D-form alanine.
  SITE 50: note = 50th amino acid(Xaa) is a 6-aminohexanoic acid.
MRGSHHHHHHGSDDDDKIVDILMQYIKANSKFIGIXXKXVAAWTLKAAXX

SEQ ID NO: 133 - protein, 78 aa, synthetic construct
  source 1..78: note = Unit peptide
  SITE 49: note = 49th amino acid(Xaa) is a 6-aminohexanoic acid.
  SITE 50: note = 50th amino acid(Xaa) is a D-form alanine.
  SITE 52: note = 52nd amino acid(Xaa) is L-cyclohexylalanins.
  SITE 62: note = 62nd amino acid(Xaa) is a D-form alanine.
  SITE 63: note = 63rd amino acid(Xaa) is a 6-aminohexanoic acid.
MRGSHHHHHHGSDDDDKIVDRNVPPIFNDVYWIAFGGGGSGGGGGGSSXXKXVAAWTLKAAXXILMQYIKANSKFIGI

SEQ ID NO: 134 - protein, 125 aa, synthetic construct
  source 1..125: note = Unit peptide
MRGSHHHHHHGSDDDDKIVDRNVPPIFNDVYWIAFGGGGSGGGGGGSSILMQYIKANSKFIGIPMGLPQSIALSSLMVAQGGGGSGGGGGGSSILMQYIKANSKFIGIPMGLPQSIALSSLMVAQ

SEQ ID NO: 135 - protein, 43 aa, synthetic construct
  source 1..43: note = Unit peptide
  SITE 16: note = 16th amino acid(Xaa) is a 6-aminohexanoic acid.
  SITE 17: note = 17th aminoacid(Xaa) is a D-form alanine.
  SITE 19: note = 19th amino acid(Xaa) is L-cyclohexylalanins.
  SITE 29: note = 29th amino acid(Xaa) is a D-form alanine.
  SITE 30: note = 30th amino acid(Xaa) is a 6-aminohexanoic acid.
  SITE 32: note = 32nd amino acid is L-cyclohexylalanins.
  SITE 42: note = 42nd amino acid(Xaa) is a D-form alanine.
  SITE 43: note = 43rd amino acid is a 6-aminohexanoic acid.
RNVPPIFNDVYWIAFXXKXVAAWTLKAAXXKXLAAFTIRAAXX

SEQ ID NO: 136 - protein, 47 aa, synthetic construct
  source 1..47: note = Unit peptide
  SITE 17: note = 17th amino acid(Xaa) is a 6-aminohexanoic acid.
  SITE 18: note = 18th amino acid(Xaa) is a D-form alanine.
  SITE 20: note = 20th amino acid(Xaa) is L-cyclohexylalanins.
  SITE 30: note = 30th amino acid(Xaa) is a D-form alanine.
  SITE 31: note = 31st amino acid(Xaa) is a 6-aminohexanoic acid.
CRNVPPIFNDVYWIAFXXKXVAAWTLKAAXXILMQYIKANSKFIGIC

SEQ ID NO: 137 - protein, 60 aa, synthetic construct
  source 1..60: note = Unit peptide
  SITE 16: note = 16th amino acid(Xaa) is a 6-aminohexanoic acid.
  SITE 17: note = 17th amino acid(Xaa) is a D-form alanine.
  SITE 19: note = 19th amino acid(Xaa) is L-cyclohexylalanins.
  SITE 29: note = 29th amino acid(Xaa) is a D-form alanine.
  SITE 30: note = 30th amino acid(Xaa) is a 6-aminohexanoic acid.
RNVPPIFNDVYWIAFXXKXVAAWTLKAAXXILMQYIKANSKFIGIRNVPPIFNDVYWIAF

SEQ ID NO: 138 - protein, 60 aa, synthetic construct
  source 1..60: note = Unit peptide
  SITE 16: note = 16th amino acid(Xaa) is a 6-aminohexanoic acid.
  SITE 17: note = 17th amino acid(Xaa) is a D-form alanine.
  SITE 19: note = 19th amino acid(Xaa) is L-cyclohexylalanins.
  SITE 29: note = 29th amino acid(Xaa) is a D-form alanine.
  SITE 30: note = 30th amino acid(Xaa) is a 6-aminohexanoic acid.
RNVPPIFNDVYWIAFXXKXVAAWTLKAAXXILMQYIKANSKFIGICRFRGLISLSQVYLS

SEQ ID NO: 139 - protein, 65 aa, synthetic construct
  source 1..65: note = Unit peptide
  SITE 16: note = 16th amino acid(Xaa) is a 6-aminohexanoic acid.
  SITE 17: note = 17th amino acid(Xaa) is a D-form alanine.
  SITE 19: note = 19th amino acid(Xaa) is L-cyclohexylalanins.
  SITE 29: note = 29th amino acid(Xaa) is a D-form alanine.
  SITE 30: note = 30th amino acid(Xaa) is a 6-aminohexanoic acid.
RNVPPIFNDVYWIAFXXKXVAAWTLKAAXXILMQYIKANSKFIGIKTTKQSFDLSVKAQYKKNKH

SEQ ID NO: 140 - protein, 60 aa, synthetic construct
  source 1..60: note = Unit peptide
  SITE 16: note = 16th amino acid(Xaa) is a 6-aminohexanoic acid.
  SITE 17: note = 17th amino acid(Xaa) is a D-form alanine.
  SITE 19: note = 19th amino acid(Xaa) is L-cyclohexylalanins.
  SITE 29: note = 29th amino acid(Xaa) is a D-form alanine.
  SITE 30: note = 30th amino acid(Xaa) is a 6-aminohexanoic acid.
CRFRGLISLSQVYLSXXKXVAAWTLKAAXXILMQYIKANSKFIGIRNVPPIFNDVYWIAF

SEQ ID NO: 141 - protein, 60 aa, synthetic construct
  source 1..60: note = Unit peptide
  SITE 16: note = 16th amino acid(Xaa) is a 6-aminohexanoic acid.
  SITE 17: note = 17th amino acid(Xaa) is a D-form alanine.
  SITE 19: note = 19th amino acid(Xaa) is L-cyclohexylalanins.
  SITE 29: note = 29th amino acid(Xaa) is a D-form alanine.
  SITE 30: note = 30th amino acid(Xaa) is a 6-aminohexanoic acid.
CRFRGLISLSQVYLSXXKXVAAWTLKAAXXILMQYIKANSKFIGICRFRGLISLSQVYLS

SEQ ID NO: 142 - protein, 65 aa, synthetic construct
  source 1..65: note = Unit peptide
  SITE 16: note = 16th amino acid(Xaa) is a 6-aminohexanoic acid.
  SITE 17: note = 17th amino acid(Xaa) is a D-form alanine.
  SITE 19: note = 19th amino acid(Xaa) is L-cyclohexylalanins.
  SITE 29: note = 29th amino acid(Xaa) is a D-form alanine.
  SITE 30: note = 30th amino acid(Xaa) is a 6-aminohexanoic acid.
CRFRGLISLSQVYLSXXKXVAAWTLKAAXXILMQYIKANSKFIGIKTTKQSFDLSVKAQYKKNKH

SEQ ID NO: 143 - protein, 65 aa, synthetic construct
  source 1..65: note = Unit peptide
  SITE 21: note = 21st amino acid(Xaa) is a 6-aminohexanoic acid.
  SITE 22: note = 22nd amino acid(Xaa) is a D-form alanine.
  SITE 24: note = 24th amino acid(Xaa) is L-cyclohexylalanins.
  SITE 34: note = 34th amino acid(Xaa) is a D-form alanine.
  SITE 35: note = 35th amino acid(Xaa) is a 6-aminohexanoic acid.
KTTKQSFDLSVKAQYKKNKHXXKXVAAWTLKAAXXILMQYIKANSKFIGIRNVPPIFNDVYWIAF

SEQ ID NO: 144 - protein, 65 aa, synthetic construct
  source 1..65: note = Unit peptide
  SITE 21: note = 21st amino acid(Xaa) is a 6-aminohexanoic acid.
  SITE 22: note = 22nd aminoacid(Xaa) is a D-form alanine.
  SITE 24: note = 24th amino acid(Xaa) isL-cyclohexylalanins.
  SITE 34: note = 34th amino acid(Xaa) is a D-form alanine.
  SITE 35: note = 35th amino acid(Xaa) is a 6-aminohexanoic acid.
KTTKQSFDLSVKAQYKKNKHXXKXVAAWTLKAAXXILMQYIKANSKFIGICRFRGLISLSQVYLS

SEQ ID NO: 145 - protein, 70 aa, synthetic construct
  source 1..70: note = Unit peptide
  SITE 21: note = 21st amino acid(Xaa) is a 6-aminohexanoic acid.
  SITE 22: note = 22nd amino acid(Xaa) is a D-form alanine.
  SITE 24: note = 24th amino acid(Xaa) is L-cyclohexylalanins.
  SITE 34: note = 34th amino acid(Xaa) is a D-form alanine.
  SITE 35: note = 35th amino acid(Xaa) is a 6-aminohexanoic acid.
KTTKQSFDLSVKAQYKKNKHXXKXVAAWTLKAAXXILMQYIKANSKFIGIKTTKQSFDLSVKAQYKKNKH

SEQ ID NO: 146 - protein, 80 aa, synthetic construct
  source 1..80: note = Unit peptide
  SITE 36: note = 36th amino acid(Xaa) is a 6-aminohexanoic acid.
  SITE 37: note = 37th amino acid(Xaa) is a D-form alanine.
  SITE 39: note = 39th amino acid(Xaa) is L-cyclohexylalanins.
  SITE 49: note = 49th amino acid(Xaa) is a D-form alanine.
  SITE 50: note = 50th amino acid(Xaa) is a 6-aminohexanoic acid.
MRGSHHHHHHGSDDDDKIVDRNVPPIFNDVYWIAFXXKXVAAWTLKAAXXILMQYIKANSKFIGIRNVPPIFNDVYWIAF

SEQ ID NO: 147 - protein, 140 aa, synthetic construct
  source 1..140: note = Unit peptide
MRGSHHHHHHGSDDDDKIVDRNVPPIFNDVYWIAFGGGGSGGGGGGSSILMQYIKANSKFIGIPMGLPQSIALSSLMVAQILMQYIKANSKFIGIPMGLPQSIALSSLMVAQGGGGSGGGGGGSSCRFRGLISLSQVYLS

SEQ ID NO: 148 - protein, 44 aa, synthetic construct
  source 1..44: note = Unit peptide
  SITE 13: note = 13rd amino acid(Xaa) is L-cyclohexylalanins.
  SITE 24: note = 24th amino acid(Xaa)is L-cyclohexylalanins.
PIFNDVYWIAFKXVAAWTLKAAKXVAAWTLKAACRFRGLISLSQ

SEQ ID NO: 149 - protein, 40 aa, synthetic construct
  source 1..40: note = Unit peptide
  SITE 11: note = 11st amino acid(Xaa) is L-cyclohexylalanins.
  SITE 22: note = 22nd amino acid(Xaa)is L-cyclohexylalanins.
PPIFNDVYWKXVAAWTLKAAKXVAAWTLKAARGLISLSQV

SEQ ID NO: 150 - protein, 62 aa, synthetic construct
  source 1..62: note = Unit peptide (cyclic)
  SITE 17: note = 17th amino acid(Xaa) is a 6-aminohexanoic acid.
  SITE 18: note = 18th amino acid(Xaa) is a D-form alanine.
  SITE 20: note = 20th amino acid(Xaa) is L-cyclohexylalanins.
  SITE 30: note = 30th amino acid(Xaa) is a D-form alanine.
  SITE 31: note = 31st amino acid(Xaa) is a 6-aminohexanoic acid.
CRNVPPIFNDVYWIAFXXKXVAAWTLKAAXXILMQYIKANSKFIGIRNVPPIFNDVYWIAFC

SEQ ID NO: 151 - protein, 80 aa, synthetic construct
  source 1..80: note = Concatamer
  SITE 36: note = Each of 36th, 50th, 66th, and 80th amino acid(Xaa) is a 6-aminohexanoic acid.
  SITE 50: note = Each of 36th, 50th, 66th, and 80th amino acid(Xaa) is a 6-aminohexanoic acid.
  SITE 66: note = Each of 36th, 50th, 66th, and 80th amino acid(Xaa) is a 6-aminohexanoic acid.
  SITE 80: note = Each of 36th, 50th, 66th, and 80th amino acid(Xaa) is a 6-aminohexanoic acid.
  SITE 37: note = Each of 37th, 49th, 67th, and 79th aminoacid(Xaa) is a D-form alanine.
  SITE 49: note = Each of 37th, 49th, 67th, and 79th aminoacid(Xaa) is a D-form alanine.
  SITE 67: note = Each of 37th, 49th, 67th, and 79th aminoacid(Xaa) is a D-form alanine.
  SITE 79: note = Each of 37th, 49th, 67th, and 79th aminoacid(Xaa) is a D-form alanine.
  SITE 39: note = Each of 39th and 69th aminoacid(Xaa) is L-cyclohexylalanins.
  SITE 69: note = Each of 39th and 69th aminoacid(Xaa) is L-cyclohexylalanins.
MRGSHHHHHHGSDDDDKIVDRNVPPIFNDVYWIAFXXKXVAAWTLKAAXXRNVPPIFNDVYWIAFXXKXVAAWTLKAAXX

SEQ ID NO: 152 - protein, 90 aa, synthetic construct
  source 1..90: note = Concatamer
  SITE 31: note = Each of 31st, 45th, 76th, and 90th amino acid(Xaa) is a 6-aminohexanoic acid.
  SITE 45: note = Each of 31st, 45th, 76th, and 90th amino acid(Xaa) is a 6-aminohexanoic acid.
  SITE 76: note = Each of 31st, 45th, 76th, and 90th amino acid(Xaa) is a 6-aminohexanoic acid.
  SITE 90: note = Each of 31st, 45th, 76th, and 90th amino acid(Xaa) is a 6-aminohexanoic acid.
  SITE 32: note = Each of 32nd, 44th, 77th, and 89th aminoacid(Xaa) is a D-form alanine.
  SITE 44: note = Each of 32nd, 44th, 77th, and 89th aminoacid(Xaa) is a D-form alanine.
  SITE 77: note = Each of 32nd, 44th, 77th, and 89th aminoacid(Xaa) is a D-form alanine.
  SITE 89: note = Each of 32nd, 44th, 77th, and 89th aminoacid(Xaa) is a D-form alanine.
  SITE 34: note = Each of 34th and 79th aminoacid(Xaa) is L-cyclohexylalanins.
  SITE 79: note = Each of 34th and 79th aminoacid(Xaa) is L-cyclohexylalanins.
RNVPPIFNDVYWIAFCRFRGLISLSQVYLSXXKXVAAWTLKAAXXRNVPPIFNDVYWIAFCRFRGLISLSQVYLSXXKXVAAWTLKAAXX

SEQ ID NO: 153 - protein, 90 aa, synthetic construct
  source 1..90: note = Concatamer
  SITE 16: note = Each of 16th, 30th, 61st, and 75th amino acid(Xaa) is a6-aminohexanoic acid.
  SITE 30: note = Each of 16th, 30th, 61st, and 75th amino acid(Xaa) is a6-aminohexanoic acid.
  SITE 61: note = Each of 16th, 30th, 61st, and 75th amino acid(Xaa) is a6-aminohexanoic acid.
  SITE 75: note = Each of 16th, 30th, 61st, and 75th amino acid(Xaa) is a6-aminohexanoic acid.
  SITE 17: note = Each of 17th, 29th, 62nd, and 74th aminoacid(Xaa) is a D-form alanine.
  SITE 29: note = Each of 17th, 29th, 62nd, and 74th aminoacid(Xaa) is a D-form alanine.
  SITE 62: note = Each of 17th, 29th, 62nd, and 74th aminoacid(Xaa) is a D-form alanine.
  SITE 74: note = Each of 17th, 29th, 62nd, and 74th aminoacid(Xaa) is a D-form alanine.
  SITE 19: note = Each of 19th and 64th aminoacid(Xaa) is L-cyclohexylalanins.
  SITE 64: note = Each of 19th and 64th aminoacid(Xaa) is L-cyclohexylalanins.
RNVPPIFNDVYWIAFXXKXVAAWTLKAAXXCRFRGLISLSQVYLSRNVPPIFNDVYWIAFXXKXVAAWTLKAAXXCRFRGLISLSQVYLS

SEQ ID NO: 154 - protein, 90 aa, synthetic construct
  source 1..90: note = Concatamer
  SITE 16: note = Each of 16th, 30th, 61st, and 75th amino acid(Xaa) is a 6-aminohexanoic acid.
  SITE 30: note = Each of 16th, 30th, 61st, and 75th amino acid(Xaa) is a 6-aminohexanoic acid.
  SITE 61: note = Each of 16th, 30th, 61st, and 75th amino acid(Xaa) is a 6-aminohexanoic acid.
  SITE 75: note = Each of 16th, 30th, 61st, and 75th amino acid(Xaa) is a 6-aminohexanoic acid.
  SITE 17: note = Each of 17th, 29th, 62nd and 74th aminoacid(Xaa) is a D-form alanine.
  SITE 29: note = Each of 17th, 29th, 62nd and 74th aminoacid(Xaa) is a D-form alanine.
  SITE 62: note = Each of 17th, 29th, 62nd and 74th aminoacid(Xaa) is a D-form alanine.
  SITE 74: note = Each of 17th, 29th, 62nd and 74th aminoacid(Xaa) is a D-form alanine.
  SITE 19: note = Each of 19th and 64th aminoacid(Xaa) is L-cyclohexylalanins.
  SITE 64: note = Each of 19th and 64th aminoacid(Xaa) is L-cyclohexylalanins.
RNVPPIFNDVYWIAFXXKXVAAWTLKAAXXILMQYIKANSKFIGIRNVPPIFNDVYWIAFXXKXVAAWTLKAAXXILMQYIKANSKFIGI

SEQ ID NO: 155 - protein, 120 aa, synthetic construct
  source 1..120: note = Concatamer
  SITE 16: note = Each of 16th, 30th, 76th, and 90th amino acid(Xaa) is a 6-aminohexanoic acid.
  SITE 30: note = Each of 16th, 30th, 76th, and 90th amino acid(Xaa) is a 6-aminohexanoic acid.
  SITE 76: note = Each of 16th, 30th, 76th, and 90th amino acid(Xaa) is a 6-aminohexanoic acid.
  SITE 90: note = Each of 16th, 30th, 76th, and 90th amino acid(Xaa) is a 6-aminohexanoic acid.
  SITE 17: note = Each of 17th, 29th, 77th, and 89th aminoacid(Xaa) is a D-form alanine.
  SITE 29: note = Each of 17th, 29th, 77th, and 89th aminoacid(Xaa) is a D-form alanine.
  SITE 29: note = Each of 17th, 29th, 77th, and 89th aminoacid(Xaa) is a D-form alanine.
  SITE 77: note = Each of 17th, 29th, 77th, and 89th aminoacid(Xaa) is a D-form alanine.
  SITE 89: note = Each of 17th, 29th, 77th, and 89th aminoacid(Xaa) is a D-form alanine.
  SITE 19: note = Each of 19th and 79th aminoacid(Xaa) is L-cyclohexylalanins.
  SITE 79: note = Each of 19th and 79th aminoacid(Xaa) is L-cyclohexylalanins.
RNVPPIFNDVYWIAFXXKXVAAWTLKAAXXILMQYIKANSKFIGIRNVPPIFNDVYWIAFRNVPPIFNDVYWIAFXXKXVAAWTLKAAXXILMQYIKANSKFIGIRNVPPIFNDVYWIAF

SEQ ID NO: 156 - protein, 75 aa, synthetic construct
  source 1..75: note = String-of-Beads
  SITE 16: note = Each of 16th, 30th, 61st, and 75th amino acid(Xaa) is a 6-aminohexanoic acid.
  SITE 30: note = Each of 16th, 30th, 61st, and 75th amino acid(Xaa) is a 6-aminohexanoic acid.
  SITE 61: note = Each of 16th, 30th, 61st, and 75th amino acid(Xaa) is a 6-aminohexanoic acid.
  SITE 75: note = Each of 16th, 30th, 61st, and 75th amino acid(Xaa) is a 6-aminohexanoic acid.
  SITE 17: note = Each of 17th, 29th, 62nd, and 74th aminoacid(Xaa) is a D-form alanine.
  SITE 29: note = Each of 17th, 29th, 62nd, and 74th aminoacid(Xaa) is a D-form alanine.
  SITE 62: note = Each of 17th, 29th, 62nd, and 74th aminoacid(Xaa) is a D-form alanine.
  SITE 74: note = Each of 17th, 29th, 62nd, and 74th aminoacid(Xaa) is a D-form alanine.
  SITE 19: note = Each of 19th and 64th aminoacid(Xaa) is L-cyclohexylalanins.
  SITE 64: note = Each of 19th and 64th aminoacid(Xaa) is L-cyclohexylalanins.
RNVPPIFNDVYWIAFXXKXVAAWTLKAAXXRNVPPIFNDVYWIAFCRFRGLISLSQVYLSXXKXVAAWTLKAAXX

SEQ ID NO: 157 - protein, 152 aa, synthetic construct
  source 1..152: note = String-of-Beads
  SITE 16: note = 16th, 30th, 46th, 62nd, 76th, 92nd, 108th, and 122nd Xaa is a 6-aminohexanoic acid.
  SITE 30: note = 16th, 30th, 46th, 62nd, 76th, 92nd, 108th, and 122nd Xaa is a 6-aminohexanoic acid.
  SITE 46: note = 16th, 30th, 46th, 62nd, 76th, 92nd, 108th, and 122nd Xaa is a 6-aminohexanoic acid.
  SITE 62: note = 16th, 30th, 46th, 62nd, 76th, 92nd, 108th, and 122nd Xaa is a 6-aminohexanoic acid.
  SITE 76: note = 16th, 30th, 46th, 62nd, 76th, 92nd, 108th, and 122nd Xaa is a 6-aminohexanoic acid.
  SITE 92: note = 16th, 30th, 46th, 62nd, 76th, 92nd, 108th, and 122nd Xaa is a 6-aminohexanoic acid.
  SITE 108: note = 16th, 30th, 46th, 62nd, 76th, 92nd, 108th, and 122nd Xaa is a 6-aminohexanoic acid.
  SITE 122: note = 16th, 30th, 46th, 62nd, 76th, 92nd, 108th, and 122nd Xaa is a 6-aminohexanoic acid.
  SITE 17: note = 17th, 29th, 63rd, 75th, 109th, and 121st Xaa is a D-form alanine.
  SITE 29: note = 17th, 29th, 63rd, 75th, 109th, and 121st Xaa is a D-form alanine.
  SITE 63: note = 17th, 29th, 63rd, 75th, 109th, and 121st Xaa is a D-form alanine.
  SITE 75: note = 17th, 29th, 63rd, 75th, 109th, and 121st Xaa is a D-form alanine.
  SITE 109: note = 17th, 29th, 63rd, 75th, 109th, and 121st Xaa is a D-form alanine.
  SITE 121: note = 17th, 29th, 63rd, 75th, 109th, and 121st Xaa is a D-form alanine.
  SITE 19: note = 19th, 65th, and 111st Xaa isL-cyclohexylalanins.
  SITE 65: note = 19th, 65th, and 111st Xaa isL-cyclohexylalanins.
  SITE 111: note = 19th, 65th, and 111st Xaa isL-cyclohexylalanins.
RNVPPIFNDVYWIAFXXKXVAAWTLKAAXXRNVPPIFNDVYWIAFXRNVPPIFNDVYWIAFXXKXVAAWTLKAAXXILMQYIKANSKFIGIXRNVPPIFNDVYWIAFXXKXVAAWTLKAAXXILMQYIKANSKFIGICRFRGLISLSQVYLS

SEQ ID NO: 158 - protein, 272 aa, synthetic construct
  source 1..272: note = String-of-Beads
  SITE 16: note = 6-aminohexanoic acid
  SITE 30: note = 6-aminohexanoic acid
  SITE 61: note = 6-aminohexanoic acid
  SITE 75: note = 6-aminohexanoic acid
  SITE 106: note = 6-aminohexanoic acid
  SITE 120: note = 6-aminohexanoic acid
  SITE 136: note = 6-aminohexanoic acid
  SITE 150: note = 6-aminohexanoic acid
  SITE 166: note = 6-aminohexanoic acid
  SITE 182: note = 6-aminohexanoic acid
  SITE 196: note = 6-aminohexanoic acid
  SITE 212: note = 6-aminohexanoic acid
  SITE 228: note = 6-aminohexanoic acid
  SITE 242: note = 6-aminohexanoic acid
  SITE 17: note = D-form alanine
  SITE 29: note = D-form alanine
  SITE 62: note = D-form alanine
  SITE 74: note = D-form alanine
  SITE 107: note = D-form alanine
  SITE 119: note = D-form alanine
  SITE 137: note = D-form alanine
  SITE 149: note = D-form alanine
  SITE 183: note = D-form alanine
  SITE 195: note = D-form alanine
  SITE 229: note = D-form alanine
  SITE 241: note = D-form alanine
  SITE 19: note = L-cyclohexylalanins
  SITE 64: note = L-cyclohexylalanins
  SITE 109: note = L-cyclohexylalanins
  SITE 139: note = L-cyclohexylalanins
  SITE 185: note = L-cyclohexylalanins
  SITE 231: note = L-cyclohexylalanins
RNVPPIFNDVYWIAFXXKXVAAWTLKAAXXRNVPPIFNDVYWIAFCRFRGLISLSQVYLSXXKXVAAWTLKAAXXRNVPPIFNDVYWIAFCRFRGLISLSQVYLSXXKXVAAWTLKAAXXRNVPPIFNDVYWIAFXXKXVAAWTLKAAXXRNVPPIFNDVYWIAFXRNVPPIFNDVYWIAFXXKXVAAWTLKAAXXILMQYIKANSKFIGIXRNVPPIFNDVYWIAFXXKXVAAWTLKAAXXILMQYIKANSKFIGICRFRGLISLSQVYLS

SEQ ID NO: 159 - protein, 6 aa, synthetic construct
  source 1..6: note = Auxiliary part
RRRRRR

SEQ ID NO: 160 - protein, 43 aa, synthetic construct
  source 1..43: note = Unit peptide
  SITE 19: note = Xaa at position 19 is L-cyclohexylalanine
  SITE 16: note = Xaa at position 16 is 6-aminohexanoic acid
  SITE 17: note = Xaa at position 17 is D-form alanine
RNVPPIFNDVYWIAFXXKXVAAWTLKAACRFRGLISLSQVYLS

SEQ ID NO: 161 - protein, 30 aa, synthetic construct
  source 1..30: note = Unit peptide
  SITE 16: note = Xaa at position 16 is 6-aminohexanoic acid
  SITE 17: note = Xaa at position 17 is D-form alanine
  SITE 19: note = Xaa at position 19 is L-cyclohexylalanine
RNVPPIFNDVYWIAFXXKXVAAWTLKAACR

SEQ ID NO: 162 - protein, 10 aa, synthetic construct
  source 1..10: note = Th epitope
PLGFFPDHQL

SEQ ID NO: 163 - protein, 16 aa, synthetic construct
  source 1..16: note = Th epitope
WPEANQVGAGAFGPGF

SEQ ID NO: 164 - protein, 15 aa, synthetic construct
  source 1..15: note = Th epitope
MQWNSTALHQALQDP

SEQ ID NO: 165 - protein, 26 aa, synthetic construct
  source 1..26: note = Th epitope
MQWNSTTFHQTLQDPRVRGLYFPAGG

SEQ ID NO: 166 - protein, 10 aa, synthetic construct
  source 1..10: note = Th epitope
FFLLTRILTI

SEQ ID NO: 167 - protein, 15 aa, synthetic construct
  source 1..15: note = Th epitope
FFLLTRILTIPQSLD

SEQ ID NO: 168 - protein, 15 aa, synthetic construct
  source 1..15: note = Th epitope
TSLNFLGGTTVCLGQ

SEQ ID NO: 169 - protein, 16 aa, synthetic construct
  source 1..16: note = Th epitope
QSPTSNHSPTSCPPIC

SEQ ID NO: 170 - protein, 19 aa, synthetic construct
  source 1..19: note = Th epitope
IIFLFILLLCLIFLLVLLD

SEQ ID NO: 171 - protein, 14 aa, synthetic construct
  source 1..14: note = Th epitope
CTTPAQGNSMFPSC

SEQ ID NO: 172 - protein, 8 aa, synthetic construct
  source 1..8: note = Th epitope
CTKPTDGN

SEQ ID NO: 173 - protein, 8 aa, synthetic construct
  source 1..8: note = Th epitope
WASVRFSW

SEQ ID NO: 174 - protein, 9 aa, synthetic construct
  source 1..9: note = Th epitope
LLPIFFCLW

SEQ ID NO: 175 - protein, 20 aa, synthetic construct
  source 1..20: note = Th epitope
MDIDPYKEFGATVELLSFLP

SEQ ID NO: 176 - protein, 10 aa, synthetic construct
  source 1..10: note = Th epitope
FLPSDFFPSV

SEQ ID NO: 177 - protein, 20 aa, synthetic construct
  source 1..20: note = Th epitope
RDLLDTASALYREALESPEH

SEQ ID NO: 178 - protein, 20 aa, synthetic construct
  source 1..20: note = Th epitope
PHHTALRQAILCWGELMTLA

SEQ ID NO: 179 - protein, 15 aa, synthetic construct
  source 1..15: note = Th epitope
GRETVIEYLVSFGVW

SEQ ID NO: 180 - protein, 15 aa, synthetic construct
  source 1..15: note = Th epitope
EYLVSFGVWIRTPPA

SEQ ID NO: 181 - protein, 20 aa, synthetic construct
  source 1..20: note = Th epitope
VSFGVWIRTPPAYRPPNAPI

SEQ ID NO: 182 - protein, 10 aa, synthetic construct
  source 1..10: note = Th epitope
TVVRRRGRSP

SEQ ID NO: 183 - protein, 15 aa, synthetic construct
  source 1..15: note = Th epitope
VGPLTVNEKRRLKLI

SEQ ID NO: 184 - protein, 15 aa, synthetic construct
  source 1..15: note = Th epitope
RHYLHTLWKAGILYK

SEQ ID NO: 185 - protein, 15 aa, synthetic construct
  source 1..15: note = Th epitope
ESRLVVDFSQFSRGN

SEQ ID NO: 186 - protein, 15 aa, synthetic construct
  source 1..15: note = Th epitope
LQSLTNLLSSNLSWL

SEQ ID NO: 187 - protein, 15 aa, synthetic construct
  source 1..15: note = Th epitope
SSNLSWLSLDVSAAF

SEQ ID NO: 188 - protein, 15 aa, synthetic construct
  source 1..15: note = Th epitope
LHLYSHPIILGFRKI

SEQ ID NO: 189 - protein, 15 aa, synthetic construct
  source 1..15: note = Th epitope
KQCFRKLPVNRPIDW

SEQ ID NO: 190 - protein, 15 aa, synthetic construct
  source 1..15: note = Th epitope
LCQVFADATPTGWGL

SEQ ID NO: 191 - protein, 15 aa, synthetic construct
  source 1..15: note = Th epitope
AANWILRGTSFVYVP

SEQ ID NO: 192 - protein, 15 aa, synthetic construct
  source 1..15: note = Th epitope
EIRLKVFVLGGCRHK

SEQ ID NO: 193 - protein, 17 aa, synthetic construct
  source 1..17: note = Auxiliary part
  SITE 16: note = Xaa at position 16 is 6-aminohexanoic acid.
  SITE 17: note = Xaa at position 17 is D-form alanine.
GSHHHHHHGSDDDDKXX

SEQ ID NO: 194 - protein, 17 aa, synthetic construct
  source 1..17: note = Auxiliary part
  SITE 1: note = Xaa at position 1 is D-form alanine.
  SITE 2: note = Xaa at position 2 is 6-aminohexanoic acid.
XXGSHHHHHHGSDDDDK

SEQ ID NO: 195 - protein, 11 aa, synthetic construct
  source 1..11: note = Th epitope
KFVAAWTLKAA

SEQ ID NO: 196 - protein, 11 aa, synthetic construct
  source 1..11: note = Th epitope
KYVAAWTLKAA

SEQ ID NO: 197 - protein, 11 aa, synthetic construct
  source 1..11: note = Th epitope
  VARIANT 2: note = Xaa can be any naturally occurring amino acid
KXVAAWTLKAA

SEQ ID NO: 198 - protein, 45 aa, synthetic construct; identical to SEQ ID NO: 108
  source 1..45: note = Unit peptide
  VARIANT 16: note = X can be any amino acid.
  VARIANT 17: note = X can be any amino acid.
  VARIANT 19: note = X can be any amino acid.
  VARIANT 29: note = X can be any amino acid.
  VARIANT 30: note = X can be any amino acid.

SEQ ID NO: 199 - protein, 45 aa, synthetic construct; identical to SEQ ID NO: 68
  source 1..45: note = Unit peptide
  VARIANT 16: note = X can be any amino acid.
  VARIANT 17: note = X can be any amino acid.
  VARIANT 19: note = X can be any amino acid.
  VARIANT 29: note = X can be any amino acid.
  VARIANT 30: note = X can be any amino acid.

SEQ ID NO: 200 - protein, 45 aa, synthetic construct; identical to SEQ ID NO: 69
  source 1..45: note = Unit peptide
  VARIANT 16: note = X can be any amino acid.
  VARIANT 17: note = X can be any amino acid.
  VARIANT 19: note = X can be any amino acid.
  VARIANT 29: note = X can be any amino acid.
  VARIANT 30: note = X can be any amino acid.

SEQ ID NO: 201 - protein, 50 aa, synthetic construct; identical to SEQ ID NO: 114
  source 1..50: note = Unit peptide
  VARIANT 21: note = X can be any amino acid.
  VARIANT 22: note = X can be any amino acid.
  VARIANT 24: note = X can be any amino acid.
  VARIANT 34: note = X can be any amino acid.
  VARIANT 35: note = X can be any amino acid.

SEQ ID NO: 202 - protein, 45 aa, synthetic construct; identical to SEQ ID NO: 84
  source 1..45: note = Unit peptide
  VARIANT 31: note = X can be any amino acid.
  VARIANT 32: note = X can be any amino acid.
  VARIANT 34: note = X can be any amino acid.
  VARIANT 44: note = X can be any amino acid.
  VARIANT 45: note = X can be any amino acid.

SEQ ID NO: 203 - protein, 45 aa, synthetic construct; identical to SEQ ID NO: 121
  source 1..45: note = Unit peptide
  VARIANT 16: note = X can be any amino acid.
  VARIANT 30: note = X can be any amino acid.

SEQ ID NO: 204 - protein, 30 aa, synthetic construct; identical to SEQ ID NO: 56
  source 1..30: note = Unit peptide
  VARIANT 16: note = X can be any amino acid.
  VARIANT 17: note = X can be any amino acid.
  VARIANT 19: note = X can be any amino acid.
  VARIANT 29: note = X can be any amino acid.
  VARIANT 30: note = X can be any amino acid.

SEQ ID NO: 205 - protein, 26 aa, synthetic construct
  source 1..26: note = Unit peptide
  VARIANT 17: note = X can be any amino acid.
RNVPPIFNDVYWIAFKXVAAWTLKAA

SEQ ID NO: 206 - protein, 32 aa, synthetic construct; identical to SEQ ID NO: 67
  source 1..32: note = Unit peptide
  VARIANT 17: note = X can be any amino acid.

SEQ ID NO: 207 - protein, 43 aa, synthetic construct; identical to SEQ ID NO: 160
  source 1..43: note = Unit peptide
  VARIANT 16: note = X can be any amino acid.
  VARIANT 17: note = X can be any amino acid.
  VARIANT 19: note = X can be any amino acid.

SEQ ID NO: 208 - protein, 30 aa, synthetic construct; identical to SEQ ID NO: 161
  source 1..30: note = Unit peptide
  VARIANT 16: note = X can be any amino acid.
  VARIANT 17: note = X can be any amino acid.
  VARIANT 19: note = X can be any amino acid.

SEQ ID NO: 209 - protein, 45 aa, synthetic construct
  source 1..45: note = Unit peptide
  VARIANT 16: note = X can be any amino acid.
  VARIANT 17: note = X can be any amino acid.
  VARIANT 29: note = X can be any amino acid.
  VARIANT 30: note = X can be any amino acid.
RNVPPIFNDVYWIAFXXKFVAAWTLKAAXXCRFRGLISLSQVYLS

SEQ ID NO: 210 - protein, 30 aa, synthetic construct
  source 1..30: note = Unit peptide
  VARIANT 16: note = X can be any amino acid.
  VARIANT 17: note = X can be any amino acid.
  VARIANT 29: note = X can be any amino acid.
  VARIANT 30: note = X can be any amino acid.
RNVPPIFNDVYWIAFXXKFVAAWTLKAAXX

SEQ ID NO: 211 - protein, 43 aa, synthetic construct
  source 1..43: note = Unit peptide
  VARIANT 16: note = X can be any amino acid.
  VARIANT 17: note = X can be any amino acid.
RNVPPIFNDVYWIAFXXKFVAAWTLKAACRFRGLISLSQVYLS

SEQ ID NO: 212 - protein, 30 aa, synthetic construct
  source 1..30: note = Unit peptide
  VARIANT 16: note = X can be any amino acid.
  VARIANT 17: note = X can be any amino acid.
RNVPPIFNDVYWIAFXXKFVAAWTLKAACR

SEQ ID NO: 213 - protein, 23 aa, synthetic construct
  source 1..23: note = Unit peptide
RNVPPIFNDVYWIAFCTKPTDGN

SEQ ID NO: 214 - protein, 24 aa, synthetic construct
  source 1..24: note = Unit peptide
RNVPPIFNDVYWIAFLLPIFFCLW

SEQ ID NO: 215 - protein, 25 aa, synthetic construct
  source 1..25: note = Unit peptide
RNVPPIFNDVYWIAFFLPSDFFPSV

SEQ ID NO: 216 - protein, 55 aa, synthetic construct
  source 1..55: note = Unit peptide
  SITE 22: note = Xaa at position 22 and position 39 are D-form alanine.
  SITE 39: note = Xaa at position 22 and position 39 are D-form alanine.
  SITE 21: note = Xaa at position 21 and position 40 are 6-aminohexanoic acid.
  SITE 40: note = Xaa at position 21 and position 40 are 6-aminohexanoic acid.
KTTKQSFDLSVKAQYKKNKHXXWPEANQVGAGAFGPGFXXCRFRGLISLSQVYLS

SEQ ID NO: 217 - protein, 59 aa, synthetic construct
  source 1..59: note = Unit peptide
  SITE 22: note = Xaa at position 22 and position 43 are D-form alanine.
  SITE 43: note = Xaa at position 22 and position 43 are D-form alanine.
  SITE 21: note = Xaa at position 21 and position 44 are 6-aminohexanoic acid.
  SITE 44: note = Xaa at position 21 and position 44 are 6-aminohexanoic acid.
KTTKQSFDLSVKAQYKKNKHXXMDIDPYKEFGATVELLSFLPXXCRFRGLISLSQVYLS

SEQ ID NO: 218 - protein, 71 aa, synthetic construct
  source 1..71: note = Unit peptide
  SITE 22: note = Xaa at position 22 and position 55 are D-form alanine.
  SITE 55: note = Xaa at position 22 and position 55 are D-form alanine.
  SITE 21: note = Xaa at position 21 and position 56 are 6-aminohexanoic acid.
  SITE 56: note = Xaa at position 21 and position 56 are 6-aminohexanoic acid.
KTTKQSFDLSVKAQYKKNKHXXILMQYIKANSKFIGIPMGLPQSIALSSLMVAQXXCRFRGLISLSQVYLS

SEQ ID NO: 219 - protein, 36 aa, synthetic construct
  source 1..36: note = Unit peptide
RNVPPIFNDVYWIAFILMQYIKANSKFIGIHHHHHH

SEQ ID NO: 220 - protein, 41 aa, synthetic construct
  source 1..41: note = Unit peptide
RNVPPIFNDVYWIAFMDIDPYKEFGATVELLSFLPHHHHHH

SEQ ID NO: 221 - protein, 15 aa, synthetic construct
  source 1..15: note = B-cell epitope
RFRGLISLSQVYLDP

SEQ ID NO: 222 - protein, 15 aa, synthetic construct
  source 1..15: note = B-cell epitope
SVCGCPVGHHDVVGL

SEQ ID NO: 223 - protein, 21 aa, synthetic construct
  source 1..21: note = Th epitope
DIEKKIAKMEKASSVFNVVNS

SEQ ID NO: 224 - protein, 16 aa, synthetic construct
  source 1..16: note = Th epitope
YSGPLKAEIAQRLEDV

SEQ ID NO: 225 - protein, 11 aa, synthetic construct
  source 1..11: note = Th epitope
  VARIANT 2: note = X can be any amino acid.
KXVKANTLKAA

SEQ ID NO: 226 - protein, 11 aa, synthetic construct
  source 1..11: note = Th epitope
  VARIANT 2: note = X can be any amino acid.
KXVKANTLKAA

SEQ ID NO: 227 - protein, 11 aa, synthetic construct
  source 1..11: note = Th epitope
  VARIANT 2: note = X can be any amino acid.
KXVKAWTLKAA

SEQ ID NO: 228 - protein, 11 aa, synthetic construct
  source 1..11: note = Th epitope
  VARIANT 2: note = X can be any amino acid.
KXVKAWTLKAA

SEQ ID NO: 229 - protein, 11 aa, synthetic construct
  source 1..11: note = Th epitope
  VARIANT 2: note = X can be any amino acid.
KXVWANTLKAA

SEQ ID NO: 230 - protein, 11 aa, synthetic construct
  source 1..11: note = Th epitope
  VARIANT 2: note = X can be any amino acid.
KXVWANTLKAA

SEQ ID NO: 231 - protein, 11 aa, synthetic construct
  source 1..11: note = Th epitope
  VARIANT 2: note = X can be any amino acid.
KXVWAYTLKAA

SEQ ID NO: 232 - protein, 11 aa, synthetic construct
  source 1..11: note = Th epitope
  VARIANT 2: note = X can be any amino acid.
KXVWAVTLKAA

SEQ ID NO: 233 - protein, 11 aa, synthetic construct
  source 1..11: note = Th epitope
  VARIANT 2: note = X can be any amino acid.
KXVYAWTLKAA

SEQ ID NO: 234 - protein, 11 aa, synthetic construct
  source 1..11: note = Th epitope
  VARIANT 2: note = X can be any amino acid.
KXVYAWTLKAA

SEQ ID NO: 235 - protein, 11 aa, synthetic construct
  source 1..11: note = Th epitope
  VARIANT 2: note = X can be any amino acid.
RXVRANTLKAA

SEQ ID NO: 236 - protein, 11 aa, synthetic construct
  source 1..11: note = Th epitope
  VARIANT 2: note = X can be any amino acid.
KXVKAHTLKAA

SEQ ID NO: 237 - protein, 11 aa, synthetic construct
  source 1..11: note = Th epitope
  VARIANT 2: note = X can be any amino acid.
KXVKAHTLKAA

SEQ ID NO: 238 - protein, 11 aa, synthetic construct
  source 1..11: note = Th epitope
  VARIANT 2: note = X can be any amino acid.
KXVAANTLKAA

SEQ ID NO: 239 - protein, 11 aa, synthetic construct
  source 1..11: note = Th epitope
  VARIANT 2: note = X can be any amino acid.
KXVAANTLKAA

SEQ ID NO: 240 - protein, 11 aa, synthetic construct
  source 1..11: note = Th epitope
  VARIANT 2: note = X can be any amino acid.
KXVAAYTLKAA

SEQ ID NO: 241 - protein, 11 aa, synthetic construct
  source 1..11: note = Th epitope
  VARIANT 2: note = X can be any amino acid.
KXVAAYTLKAA

SEQ ID NO: 242 - protein, 11 aa, synthetic construct
  source 1..11: note = Th epitope
  VARIANT 2: note = X can be any amino acid.
KXVAAWTLKAA

SEQ ID NO: 243 - protein, 11 aa, synthetic construct
  source 1..11: note = Th epitope
  VARIANT 2: note = X can be any amino acid.
KXVAAKTLKAA

SEQ ID NO: 244 - protein, 11 aa, synthetic construct
  source 1..11: note = Th epitope
  VARIANT 2: note = X can be any amino acid.
KXVAAHTLKAA

SEQ ID NO: 245 - protein, 11 aa, synthetic construct
  source 1..11: note = Th epitope
  VARIANT 2: note = X can be any amino acid.
KXVAAATLKAA

SEQ ID NO: 246 - protein, 11 aa, synthetic construct
  source 1..11: note = Th epitope
  VARIANT 2: note = X can be any amino acid.
KXVAAWTLKAA

SEQ ID NO: 247 - protein, 11 aa, synthetic construct
  source 1..11: note = Th epitope
  VARIANT 2: note = X can be any amino acid.
KXVMAATLKAA

SEQ ID NO: 248 - DNA, 135 bp, synthetic construct
  source 1..135: mol_type = other DNA; note = DNA encoding unit peptide
cgtaatgttcctcctatcttcaatgatgtttattggattgcattcnnnnnnaagnnngtggcagcttggaccctgaaggcagcannnnnntgccgtttccgtggactgatttccctgtcccaggtttatctgtcc

SEQ ID NO: 249 - DNA, 135 bp, synthetic construct
  source 1..135: mol_type = other DNA; note = DNA encoding unit peptide
cgtaatgttcctcctatcttcaatgatgtttattggattgcattcnnnnnnaagttcgtggcagcttggaccctgaaggcagcannnnnntgccgtttccgtggactgatttccctgtcccaggtttatctgtcc

SEQ ID NO: 250 - DNA, 135 bp, synthetic construct
  source 1..135: mol_type = other DNA; note = DNA encoding unit peptide
cgtaatgttcctcctatcttcaatgatgtttattggattgcattcnnnnnnaagtatgtggcagcttggaccctgaaggcagcannnnnntgccgtttccgtggactgatttccctgtcccaggtttatctgtcc

SEQ ID NO: 251 - DNA, 135 bp, synthetic construct
  source 1..135: mol_type = other DNA; note = DNA encoding unit peptide
cgtaatgttcctcctatcttcaatgatgtttattggattgcattcnnnnnnaagnnngtggcagcttggaccctgaaggcagcannnnnnggatcgcatcaccatcaccatcacggatccgatgatgatgacaag

SEQ ID NO: 252 - DNA, 135 bp, synthetic construct
  source 1..135: mol_type = other DNA; note = DNA encoding unit peptide
cgtaatgttcctcctatcttcaatgatgtttattggattgcattcnnnnnnaagttcgtggcagcttggaccctgaaggcagcannnnnnggatcgcatcaccatcaccatcacggatccgatgatgatgacaag

SEQ ID NO: 253 - DNA, 135 bp, synthetic construct
  source 1..135: mol_type = other DNA; note = DNA encoding unit peptide
cgtaatgttcctcctatcttcaatgatgtttattggattgcattcnnnnnnaagtatgtggcagcttggaccctgaaggcagcannnnnnggatcgcatcaccatcaccatcacggatccgatgatgatgacaag

SEQ ID NO: 254 - DNA, 135 bp, synthetic construct
  source 1..135: mol_type = other DNA; note = DNA encoding unit peptide
ggatcgcatcaccatcaccatcacggatccgatgatgatgacaagnnnnnnaagnnngtggcagcttggaccctgaaggcagcannnnnncgtaatgttcctcctatcttcaatgatgtttattggattgcattc

SEQ ID NO: 255 - DNA, 135 bp, synthetic construct
  source 1..135: mol_type = other DNA; note = DNA encoding unit peptide
ggatcgcatcaccatcaccatcacggatccgatgatgatgacaagnnnnnnaagttcgtggcagcttggaccctgaaggcagcannnnnncgtaatgttcctcctatcttcaatgatgtttattggattgcattc

SEQ ID NO: 256 - DNA, 135 bp, synthetic construct
  source 1..135: mol_type = other DNA; note = DNA encoding unit peptide
ggatcgcatcaccatcaccatcacggatccgatgatgatgacaagnnnnnnaagtatgtggcagcttggaccctgaaggcagcannnnnncgtaatgttcctcctatcttcaatgatgtttattggattgcattc

SEQ ID NO: 257 - DNA, 135 bp, synthetic construct
  source 1..135: mol_type = other DNA; note = DNA encoding unit peptide
aaaacgacaaagcaatcatttgatttaagtgtaaaagctcagtatnnnnnnaagnnngtggcagcttggaccctgaaggcagcannnnnntgccgtttccgtggactgatttccctgtcccaggtttatctgtcc

SEQ ID NO: 258 - DNA, 135 bp, synthetic construct
  source 1..135: mol_type = other DNA; note = DNA encoding unit peptide
aaaacgacaaagcaatcatttgatttaagtgtaaaagctcagtatnnnnnnaagttcgtggcagcttggaccctgaaggcagcannnnnntgccgtttccgtggactgatttccctgtcccaggtttatctgtcc

SEQ ID NO: 259 - DNA, 135 bp, synthetic construct
  source 1..135: mol_type = other DNA; note = DNA encoding unit peptide
aaaacgacaaagcaatcatttgatttaagtgtaaaagctcagtatnnnnnnaagtatgtggcagcttggaccctgaaggcagcannnnnntgccgtttccgtggactgatttccctgtcccaggtttatctgtcc

SEQ ID NO: 260 - DNA, 135 bp, synthetic construct
  source 1..135: mol_type = other DNA; note = DNA encoding unit peptide
cgtaatgttcctcctatcttcaatgatgtttattggattgcattctgccgtttccgtggactgatttccctgtcccaggtttatctgtccnnnnnnaagnnngtggcagcttggaccctgaaggcagcannnnnn

SEQ ID NO: 261 - DNA, 135 bp, synthetic construct
  source 1..135: mol_type = other DNA; note = DNA encoding unit peptide
cgtaatgttcctcctatcttcaatgatgtttattggattgcattctgccgtttccgtggactgatttccctgtcccaggtttatctgtccnnnnnnaagttcgtggcagcttggaccctgaaggcagcannnnnn

SEQ ID NO: 262 - DNA, 135 bp, synthetic construct
  source 1..135: mol_type = other DNA; note = DNA encoding unit peptide
cgtaatgttcctcctatcttcaatgatgtttattggattgcattctgccgtttccgtggactgatttccctgtcccaggtttatctgtccnnnnnnaagtatgtggcagcttggaccctgaaggcagcannnnnn

SEQ ID NO: 263 - DNA, 135 bp, synthetic construct
  source 1..135: mol_type = other DNA; note = DNA encoding unit peptide
cgtaatgttcctcctatcttcaatgatgtttattggattgcattcnnncctaagtatgtgaagcagaatacactgaagctggcaaccnnntgccgtttccgtggactgatttccctgtcccaggtttatctgtcc

SEQ ID NO: 264 - DNA, 90 bp, synthetic construct
  source 1..90: mol_type = other DNA; note = DNA encoding unit peptide
cgtaatgttcctcctatcttcaatgatgtttattggattgcattcnnnnnnaagnnngtggcagcttggaccctgaaggcagcannnnnn

SEQ ID NO: 265 - DNA, 90 bp, synthetic construct
  source 1..90: mol_type = other DNA; note = DNA encoding unit peptide
cgtaatgttcctcctatcttcaatgatgtttattggattgcattcnnnnnnaagttcgtggcagcttggaccctgaaggcagcannnnnn

SEQ ID NO: 266 - DNA, 90 bp, synthetic construct
  source 1..90: mol_type = other DNA; note = DNA encoding unit peptide
cgtaatgttcctcctatcttcaatgatgtttattggattgcattcnnnnnnaagtatgtggcagcttggaccctgaaggcagcannnnnn

SEQ ID NO: 267 - DNA, 78 bp, synthetic construct
  source 1..78: mol_type = other DNA; note = DNA encoding unit peptide
cgtaatgttcctcctatcttcaatgatgtttattggattgcattcaagnnngtggcagcttggaccctgaaggcagca

SEQ ID NO: 268 - DNA, 78 bp, synthetic construct
  source 1..78: mol_type = other DNA; note = DNA encoding unit peptide
cgtaatgttcctcctatcttcaatgatgtttattggattgcattcaagttcgtggcagcttggaccctgaaggcagca

SEQ ID NO: 269 - DNA, 78 bp, synthetic construct
  source 1..78: mol_type = other DNA; note = DNA encoding unit peptide
cgtaatgttcctcctatcttcaatgatgtttattggattgcattcaagtatgtggcagcttggaccctgaaggcagca

SEQ ID NO: 270 - DNA, 96 bp, synthetic construct
  source 1..96: mol_type = other DNA; note = DNA encoding unit peptide
cgtaatgttcctcctatcttcaatgatgtttattggattgcattcaagnnngtggcagcttggaccctgaaggcagcacatcaccatcaccatcac

SEQ ID NO: 271 - DNA, 96 bp, synthetic construct
  source 1..96: mol_type = other DNA; note = DNA encoding unit peptide
cgtaatgttcctcctatcttcaatgatgtttattggattgcattcaagttcgtggcagcttggaccctgaaggcagcacatcaccatcaccatcac

SEQ ID NO: 272 - DNA, 96 bp, synthetic construct
  source 1..96: mol_type = other DNA; note = DNA encoding unit peptide
cgtaatgttcctcctatcttcaatgatgtttattggattgcattcaagtatgtggcagcttggaccctgaaggcagcacatcaccatcaccatcac

SEQ ID NO: 273 - DNA, 129 bp, synthetic construct
  source 1..129: mol_type = other DNA; note = DNA encoding unit peptide
cgtaatgttcctcctatcttcaatgatgtttattggattgcattcnnnnnnaagnnngtggcagcttggaccctgaaggcagcatgccgtttccgtggactgatttccctgtcccaggtttatctgtcc

SEQ ID NO: 274 - DNA, 129 bp, synthetic construct
  source 1..129: mol_type = other DNA; note = DNA encoding unit peptide
cgtaatgttcctcctatcttcaatgatgtttattggattgcattcnnnnnnaagttcgtggcagcttggaccctgaaggcagcatgccgtttccgtggactgatttccctgtcccaggtttatctgtcc

SEQ ID NO: 275 - DNA, 129 bp, synthetic construct
  source 1..129: mol_type = other DNA; note = DNA encoding unit peptide
cgtaatgttcctcctatcttcaatgatgtttattggattgcattcnnnnnnaagtatgtggcagcttggaccctgaaggcagcatgccgtttccgtggactgatttccctgtcccaggtttatctgtcc

SEQ ID NO: 276 - DNA, 90 bp, synthetic construct
  source 1..90: mol_type = other DNA; note = DNA encoding unit peptide
cgtaatgttcctcctatcttcaatgatgtttattggattgcattcnnnnnnaagnnngtggcagcttggaccctgaaggcagcatgccgt

SEQ ID NO: 277 - DNA, 90 bp, synthetic construct
  source 1..90: mol_type = other DNA; note = DNA encoding unit peptide
cgtaatgttcctcctatcttcaatgatgtttattggattgcattcnnnnnnaagttcgtggcagcttggaccctgaaggcagcatgccgt

SEQ ID NO: 278 - DNA, 90 bp, synthetic construct
  source 1..90: mol_type = other DNA; note = DNA encoding unit peptide
cgtaatgttcctcctatcttcaatgatgtttattggattgcattcnnnnnnaagtatgtggcagcttggaccctgaaggcagcatgccgt

SEQ ID NO: 279 - RNA, 135 nt, synthetic construct
  source 1..135: mol_type = other RNA; note = RNA encoding unit peptide
cgtaatgttcctcctatcttcaatgatgtttattggattgcattcnnnnnnaagnnngtggcagcttggaccctgaaggcagcannnnnntgccgtttccgtggactgatttccctgtcccaggtttatctgtcc

SEQ ID NO: 280 - RNA, 135 nt, synthetic construct
  source 1..135: mol_type = other RNA; note = RNA encoding unit peptide
cgtaatgttcctcctatcttcaatgatgtttattggattgcattcnnnnnnaagttcgtggcagcttggaccctgaaggcagcannnnnntgccgtttccgtggactgatttccctgtcccaggtttatctgtcc

SEQ ID NO: 281 - RNA, 135 nt, synthetic construct
  source 1..135: mol_type = other RNA; note = RNA encoding unit peptide
cgtaatgttcctcctatcttcaatgatgtttattggattgcattcnnnnnnaagtatgtggcagcttggaccctgaaggcagcannnnnntgccgtttccgtggactgatttccctgtcccaggtttatctgtcc

SEQ ID NO: 282 - RNA, 135 nt, synthetic construct
  source 1..135: mol_type = other RNA; note = RNA encoding unit peptide
cgtaatgttcctcctatcttcaatgatgtttattggattgcattcnnnnnnaagnnngtggcagcttggaccctgaaggcagcannnnnnggatcgcatcaccatcaccatcacggatccgatgatgatgacaag

SEQ ID NO: 283 - RNA, 135 nt, synthetic construct
  source 1..135: mol_type = other RNA; note = RNA encoding unit peptide
cgtaatgttcctcctatcttcaatgatgtttattggattgcattcnnnnnnaagttcgtggcagcttggaccctgaaggcagcannnnnnggatcgcatcaccatcaccatcacggatccgatgatgatgacaag

SEQ ID NO: 284 - RNA, 135 nt, synthetic construct
  source 1..135: mol_type = other RNA; note = RNA encoding unit peptide
cgtaatgttcctcctatcttcaatgatgtttattggattgcattcnnnnnnaagtatgtggcagcttggaccctgaaggcagcannnnnnggatcgcatcaccatcaccatcacggatccgatgatgatgacaag

SEQ ID NO: 285 - RNA, 135 nt, synthetic construct
  source 1..135: mol_type = other RNA; note = RNA encoding unit peptide
ggatcgcatcaccatcaccatcacggatccgatgatgatgacaagnnnnnnaagnnngtggcagcttggaccctgaaggcagcannnnnncgtaatgttcctcctatcttcaatgatgtttattggattgcattc

SEQ ID NO: 286 - RNA, 135 nt, synthetic construct
  source 1..135: mol_type = other RNA; note = RNA encoding unit peptide
ggatcgcatcaccatcaccatcacggatccgatgatgatgacaagnnnnnnaagttcgtggcagcttggaccctgaaggcagcannnnnncgtaatgttcctcctatcttcaatgatgtttattggattgcattc

SEQ ID NO: 287 - RNA, 135 nt, synthetic construct
  source 1..135: mol_type = other RNA; note = RNA encoding unit peptide
ggatcgcatcaccatcaccatcacggatccgatgatgatgacaagnnnnnnaagtatgtggcagcttggaccctgaaggcagcannnnnncgtaatgttcctcctatcttcaatgatgtttattggattgcattc

SEQ ID NO: 288 - RNA, 135 nt, synthetic construct
  source 1..135: mol_type = other RNA; note = RNA encoding unit peptide
aaaacgacaaagcaatcatttgatttaagtgtaaaagctcagtatnnnnnnaagnnngtggcagcttggaccctgaaggcagcannnnnntgccgtttccgtggactgatttccctgtcccaggtttatctgtcc

SEQ ID NO: 289 - RNA, 135 nt, synthetic construct
  source 1..135: mol_type = other RNA; note = RNA encoding unit peptide
aaaacgacaaagcaatcatttgatttaagtgtaaaagctcagtatnnnnnnaagttcgtggcagcttggaccctgaaggcagcannnnnntgccgtttccgtggactgatttccctgtcccaggtttatctgtcc

SEQ ID NO: 290 - RNA, 135 nt, synthetic construct
  source 1..135: mol_type = other RNA; note = RNA encoding unit peptide
aaaacgacaaagcaatcatttgatttaagtgtaaaagctcagtatnnnnnnaagtatgtggcagcttggaccctgaaggcagcannnnnntgccgtttccgtggactgatttccctgtcccaggtttatctgtcc

SEQ ID NO: 291 - RNA, 135 nt, synthetic construct
  source 1..135: mol_type = other RNA; note = RNA encoding unit peptide
cgtaatgttcctcctatcttcaatgatgtttattggattgcattctgccgtttccgtggactgatttccctgtcccaggtttatctgtccnnnnnnaagnnngtggcagcttggaccctgaaggcagcannnnnn

SEQ ID NO: 292 - RNA, 135 nt, synthetic construct
  source 1..135: mol_type = other RNA; note = RNA encoding unit peptide
cgtaatgttcctcctatcttcaatgatgtttattggattgcattctgccgtttccgtggactgatttccctgtcccaggtttatctgtccnnnnnnaagttcgtggcagcttggaccctgaaggcagcannnnnn

SEQ ID NO: 293 - RNA, 135 nt, synthetic construct
  source 1..135: mol_type = other RNA; note = RNA encoding unit peptide
cgtaatgttcctcctatcttcaatgatgtttattggattgcattctgccgtttccgtggactgatttccctgtcccaggtttatctgtccnnnnnnaagtatgtggcagcttggaccctgaaggcagcannnnnn

SEQ ID NO: 294 - RNA, 135 nt, synthetic construct
  source 1..135: mol_type = other RNA; note = RNA encoding unit peptide
cgtaatgttcctcctatcttcaatgatgtttattggattgcattcnnncctaagtatgtgaagcagaatacactgaagctggcaaccnnntgccgtttccgtggactgatttccctgtcccaggtttatctgtcc

SEQ ID NO: 295 - RNA, 90 nt, synthetic construct
  source 1..90: mol_type = other RNA; note = RNA encoding unit peptide
cgtaatgttcctcctatcttcaatgatgtttattggattgcattcnnnnnnaagnnngtggcagcttggaccctgaaggcagcannnnnn

SEQ ID NO: 296 - RNA, 90 nt, synthetic construct
  source 1..90: mol_type = other RNA; note = RNA encoding unit peptide
cgtaatgttcctcctatcttcaatgatgtttattggattgcattcnnnnnnaagttcgtggcagcttggaccctgaaggcagcannnnnn

SEQ ID NO: 297 - RNA, 90 nt, synthetic construct
  source 1..90: mol_type = other RNA; note = RNA encoding unit peptide
cgtaatgttcctcctatcttcaatgatgtttattggattgcattcnnnnnnaagtatgtggcagcttggaccctgaaggcagcannnnnn

SEQ ID NO: 298 - RNA, 78 nt, synthetic construct
  source 1..78: mol_type = other RNA; note = RNA encoding unit peptide
cgtaatgttcctcctatcttcaatgatgtttattggattgcattcaagnnngtggcagcttggaccctgaaggcagca

SEQ ID NO: 299 - RNA, 78 nt, synthetic construct
  source 1..78: mol_type = other RNA; note = RNA encoding unit peptide
cgtaatgttcctcctatcttcaatgatgtttattggattgcattcaagttcgtggcagcttggaccctgaaggcagca

SEQ ID NO: 300 - RNA, 78 nt, synthetic construct
  source 1..78: mol_type = other RNA; note = RNA encoding unit peptide
cgtaatgttcctcctatcttcaatgatgtttattggattgcattcaagtatgtggcagcttggaccctgaaggcagca

SEQ ID NO: 301 - RNA, 96 nt, synthetic construct
  source 1..96: mol_type = other RNA; note = RNA encoding unit peptide
cgtaatgttcctcctatcttcaatgatgtttattggattgcattcaagnnngtggcagcttggaccctgaaggcagcacatcaccatcaccatcac

SEQ ID NO: 302 - RNA, 96 nt, synthetic construct
  source 1..96: mol_type = other RNA; note = RNA encoding unit peptide
cgtaatgttcctcctatcttcaatgatgtttattggattgcattcaagttcgtggcagcttggaccctgaaggcagcacatcaccatcaccatcac

SEQ ID NO: 303 - RNA, 96 nt, synthetic construct
  source 1..96: mol_type = other RNA; note = RNA encoding unit peptide
cgtaatgttcctcctatcttcaatgatgtttattggattgcattcaagtatgtggcagcttggaccctgaaggcagcacatcaccatcaccatcac

SEQ ID NO: 304 - RNA, 129 nt, synthetic construct
  source 1..129: mol_type = other RNA; note = RNA encoding unit peptide
cgtaatgttcctcctatcttcaatgatgtttattggattgcattcnnnnnnaagnnngtggcagcttggaccctgaaggcagcatgccgtttccgtggactgatttccctgtcccaggtttatctgtcc

SEQ ID NO: 305 - RNA, 129 nt, synthetic construct
  source 1..129: mol_type = other RNA; note = RNA encoding unit peptide
cgtaatgttcctcctatcttcaatgatgtttattggattgcattcnnnnnnaagttcgtggcagcttggaccctgaaggcagcatgccgtttccgtggactgatttccctgtcccaggtttatctgtcc

SEQ ID NO: 306 - RNA, 129 nt, synthetic construct
  source 1..129: mol_type = other RNA; note = RNA encoding unit peptide
cgtaatgttcctcctatcttcaatgatgtttattggattgcattcnnnnnnaagtatgtggcagcttggaccctgaaggcagcatgccgtttccgtggactgatttccctgtcccaggtttatctgtcc

SEQ ID NO: 307 - RNA, 90 nt, synthetic construct
  source 1..90: mol_type = other RNA; note = RNA encoding unit peptide
cgtaatgttcctcctatcttcaatgatgtttattggattgcattcnnnnnnaagnnngtggcagcttggaccctgaaggcagcatgccgt

SEQ ID NO: 308 - RNA, 90 nt, synthetic construct
  source 1..90: mol_type = other RNA; note = RNA encoding unit peptide
cgtaatgttcctcctatcttcaatgatgtttattggattgcattcnnnnnnaagttcgtggcagcttggaccctgaaggcagcatgccgt

SEQ ID NO: 309 - RNA, 90 nt, synthetic construct
  source 1..90: mol_type = other RNA; note = RNA encoding unit peptide
cgtaatgttcctcctatcttcaatgatgtttattggattgcattcnnnnnnaagtatgtggcagcttggaccctgaaggcagcatgccgt